European Patent Application EP 4 516 899 A2, published March 5, 2025. Title: Nuclease having improved salt tolerance and/or temperature performance. Applicant: c-LEcta GmbH. The sequence listing filed with the application follows.

SEQUENCE LISTING (195 sequences)

SEQ ID NO: 1 - protein, 245 aa, Serratia marcescens
DTLESIDNCAVGCPTGGSSNVSIVRHAYTLNNNSTTKFANWVAYHITKDTPASGKTRNWKTDPALNPADTLAPADYTGANAALKVDRGHQAPLASLAGVSDWESLNYLSNITPQKSDLNQGAWARLEDQERKLIDRADISSVYTVTGPLYERDMGKLPGTQKAHTIPSAYWKVIFINNSPAVNHYAAFLFDQNTPKGADFCQFRVTVDEIEKRTGLIIWAGLPDDVQASLKSKPGVLPELMGCKN

SEQ ID NO: 2 - protein, 245 aa, synthetic construct
  REGION 1..245: note = isolated from library
DTLESIDNCAVGCPTGGSSNVSIVRHAYTLNNNSTTKFANWVAYHITKDTLASGKTRNWKTDPALNPADTLAPADYTGANAALKVDRGHQAPLASLAGVSDWESLNYLSNITPQKSDLNQGAWARLEDQERKLIDRADISSVYTVTGPLYERDMGKLPGTQKAHTIPSAYWKVIFINNSPAVNHYAAFLFDQNTPKGADFCQFRVTVDEIEKRTGLIIWAGLPDDVQASLKSKPGVLPELMGCKN

SEQ ID NO: 3 - protein, 245 aa, synthetic construct
  REGION 1..245: note = isolated from library
DTLESIDNCAVGCPTGGSSNVSIVRHAYTLNNNSTTKFANWVAYHITKDTRASGKTRNWKTDPALNPADTLAPADYTGANAALKVDRGHQAPLASLAGVSDWESLNYLSNITPQKSDLNQGAWARLEDQERKLIDRADISSVYTVTGPLYERDMGKLPGTQKAHTIPSAYWKVIFINNSPAVNHYAAFLFDQNTPKGADFCQFRVTVDEIEKRTGLIIWAGLPDDVQASLKSKPGVLPELMGCKN

SEQ ID NO: 4 - protein, 245 aa, synthetic construct
  REGION 1..245: note = isolated from library
DTLESIDNCAVGCPTGGSSNVSIVRHAYTLNNNSTTKFANWVAYHITKDTGASGKTRNWKTDPALNPADTLAPADYTGANAALKVDRGHQAPLASLAGVSDWESLNYLSNITPQKSDLNQGAWARLEDQERKLIDRADISSVYTVTGPLYERDMGKLPGTQKAHTIPSAYWKVIFINNSPAVNHYAAFLFDQNTPKGADFCQFRVTVDEIEKRTGLIIWAGLPDDVQASLKSKPGVLPELMGCKN

SEQ ID NO: 5 - protein, 245 aa, synthetic construct
  REGION 1..245: note = isolated from library
DTLESIDNCAVGCPTGGSSNVSIVRHAYTLNNNSTTKFANWVAYHITKDTDASGKTRNWKTDPALNPADTLAPADYTGANAALKVDRGHQAPLASLAGVSDWESLNYLSNITPQKSDLNQGAWARLEDQERKLIDRADISSVYTVTGPLYERDMGKLPGTQKAHTIPSAYWKVIFINNSPAVNHYAAFLFDQNTPKGADFCQFRVTVDEIEKRTGLIIWAGLPDDVQASLKSKPGVLPELMGCKN

SEQ ID NO: 6 - protein, 245 aa, synthetic construct
  REGION 1..245: note = isolated from library
DTLESIDNCAVGCPTGGSSNVSIVRHAYTLNNNSTTKFANWVAYHITKDTPAKGKTRNWKTDPALNPADTLAPADYTGANAALKVDRGHQAPLASLAGVSDWESLNYLSNITPQKSDLNQGAWARLEDQERKLIDRADISSVYTVTGPLYERDMGKLPGTQKAHTIPSAYWKVIFINNSPAVNHYAAFLFDQNTPKGADFCQFRVTVDEIEKRTGLIIWAGLPDDVQASLKSKPGVLPELMGCKN

SEQ ID NO: 7 - protein, 245 aa, synthetic construct
  REGION 1..245: note = isolated from library
DTLESIDNCAVGCPTGGSSNVSIVRHAYTLNNNSTTKFANWVAYHITKDTPAAGKTRNWKTDPALNPADTLAPADYTGANAALKVDRGHQAPLASLAGVSDWESLNYLSNITPQKSDLNQGAWARLEDQERKLIDRADISSVYTVTGPLYERDMGKLPGTQKAHTIPSAYWKVIFINNSPAVNHYAAFLFDQNTPKGADFCQFRVTVDEIEKRTGLIIWAGLPDDVQASLKSKPGVLPELMGCKN

SEQ ID NO: 8 - protein, 245 aa, synthetic construct
  REGION 1..245: note = isolated from library
DTLESIDNCAVGCPTGGSSNVSIVRHAYTLNNNSTTKFANWVAYHITKDTPASGRTRNWKTDPALNPADTLAPADYTGANAALKVDRGHQAPLASLAGVSDWESLNYLSNITPQKSDLNQGAWARLEDQERKLIDRADISSVYTVTGPLYERDMGKLPGTQKAHTIPSAYWKVIFINNSPAVNHYAAFLFDQNTPKGADFCQFRVTVDEIEKRTGLIIWAGLPDDVQASLKSKPGVLPELMGCKN

SEQ ID NO: 9 - protein, 245 aa, synthetic construct
  REGION 1..245: note = isolated from library
DTLESIDNCAVGCPTGGSSNVSIVRHAYTLNNNSTTKFANWVAYHITKDTPASGKPRNWKTDPALNPADTLAPADYTGANAALKVDRGHQAPLASLAGVSDWESLNYLSNITPQKSDLNQGAWARLEDQERKLIDRADISSVYTVTGPLYERDMGKLPGTQKAHTIPSAYWKVIFINNSPAVNHYAAFLFDQNTPKGADFCQFRVTVDEIEKRTGLIIWAGLPDDVQASLKSKPGVLPELMGCKN

SEQ ID NO: 10 - protein, 245 aa, synthetic construct
  REGION 1..245: note = isolated from library
DTLESIDNCAVGCPTGGSSNVSIVRHAYTLNNNSTTKFANWVAYHITKDTPASGKDRNWKTDPALNPADTLAPADYTGANAALKVDRGHQAPLASLAGVSDWESLNYLSNITPQKSDLNQGAWARLEDQERKLIDRADISSVYTVTGPLYERDMGKLPGTQKAHTIPSAYWKVIFINNSPAVNHYAAFLFDQNTPKGADFCQFRVTVDEIEKRTGLIIWAGLPDDVQASLKSKPGVLPELMGCKN

SEQ ID NO: 11 - protein, 245 aa, synthetic construct
  REGION 1..245: note = isolated from library
DTLESIDNCAVGCPTGGSSNVSIVRHAYTLNNNSTTKFANWVAYHITKDTPASGKRRNWKTDPALNPADTLAPADYTGANAALKVDRGHQAPLASLAGVSDWESLNYLSNITPQKSDLNQGAWARLEDQERKLIDRADISSVYTVTGPLYERDMGKLPGTQKAHTIPSAYWKVIFINNSPAVNHYAAFLFDQNTPKGADFCQFRVTVDEIEKRTGLIIWAGLPDDVQASLKSKPGVLPELMGCKN

SEQ ID NO: 12 - protein, 245 aa, synthetic construct
  REGION 1..245: note = isolated from library
DTLESIDNCAVGCPTGGSSNVSIVRHAYTLNNNSTTKFANWVAYHITKDTPASGKKRNWKTDPALNPADTLAPADYTGANAALKVDRGHQAPLASLAGVSDWESLNYLSNITPQKSDLNQGAWARLEDQERKLIDRADISSVYTVTGPLYERDMGKLPGTQKAHTIPSAYWKVIFINNSPAVNHYAAFLFDQNTPKGADFCQFRVTVDEIEKRTGLIIWAGLPDDVQASLKSKPGVLPELMGCKN

SEQ ID NO: 13 - protein, 245 aa, synthetic construct
  REGION 1..245: note = isolated from library
DTLESIDNCAVGCPTGGSSNVSIVRHAYTLNNNSTTKFANWVAYHITKDTPASGKTRVWKTDPALNPADTLAPADYTGANAALKVDRGHQAPLASLAGVSDWESLNYLSNITPQKSDLNQGAWARLEDQERKLIDRADISSVYTVTGPLYERDMGKLPGTQKAHTIPSAYWKVIFINNSPAVNHYAAFLFDQNTPKGADFCQFRVTVDEIEKRTGLIIWAGLPDDVQASLKSKPGVLPELMGCKN

SEQ ID NO: 14 - protein, 245 aa, synthetic construct
  REGION 1..245: note = isolated from library
DTLESIDNCAVGCPTGGSSNVSIVRHAYTLNNNSTTKFANWVAYHITKDTPASGKTRRWKTDPALNPADTLAPADYTGANAALKVDRGHQAPLASLAGVSDWESLNYLSNITPQKSDLNQGAWARLEDQERKLIDRADISSVYTVTGPLYERDMGKLPGTQKAHTIPSAYWKVIFINNSPAVNHYAAFLFDQNTPKGADFCQFRVTVDEIEKRTGLIIWAGLPDDVQASLKSKPGVLPELMGCKN

SEQ ID NO: 15 - protein, 245 aa, synthetic construct
  REGION 1..245: note = isolated from library
DTLESIDNCAVGCPTGGSSNVSIVRHAYTLNNNSTTKFANWVAYHITKDTPASGKTRKWKTDPALNPADTLAPADYTGANAALKVDRGHQAPLASLAGVSDWESLNYLSNITPQKSDLNQGAWARLEDQERKLIDRADISSVYTVTGPLYERDMGKLPGTQKAHTIPSAYWKVIFINNSPAVNHYAAFLFDQNTPKGADFCQFRVTVDEIEKRTGLIIWAGLPDDVQASLKSKPGVLPELMGCKN

SEQ ID NO: 16 - protein, 245 aa, synthetic construct
  REGION 1..245: note = isolated from library
DTLESIDNCAVGCPTGGSSNVSIVRHAYTLNNNSTTKFANWVAYHITKDTPASGKTRNWKTDPALNPADTLKPADYTGANAALKVDRGHQAPLASLAGVSDWESLNYLSNITPQKSDLNQGAWARLEDQERKLIDRADISSVYTVTGPLYERDMGKLPGTQKAHTIPSAYWKVIFINNSPAVNHYAAFLFDQNTPKGADFCQFRVTVDEIEKRTGLIIWAGLPDDVQASLKSKPGVLPELMGCKN

SEQ ID NO: 17 - protein, 245 aa, synthetic construct
  REGION 1..245: note = isolated from library
DTLESIDNCAVGCPTGGSSNVSIVRHAYTLNNNSTTKFANWVAYHITKDTPASGKTRNWKTDPALNPADTLAKADYTGANAALKVDRGHQAPLASLAGVSDWESLNYLSNITPQKSDLNQGAWARLEDQERKLIDRADISSVYTVTGPLYERDMGKLPGTQKAHTIPSAYWKVIFINNSPAVNHYAAFLFDQNTPKGADFCQFRVTVDEIEKRTGLIIWAGLPDDVQASLKSKPGVLPELMGCKN

SEQ ID NO: 18 - protein, 245 aa, synthetic construct
  REGION 1..245: note = isolated from library
DTLESIDNCAVGCPTGGSSNVSIVRHAYTLNNNSTTKFANWVAYHITKDTPASGKTRNWKTDPALNPADTLARADYTGANAALKVDRGHQAPLASLAGVSDWESLNYLSNITPQKSDLNQGAWARLEDQERKLIDRADISSVYTVTGPLYERDMGKLPGTQKAHTIPSAYWKVIFINNSPAVNHYAAFLFDQNTPKGADFCQFRVTVDEIEKRTGLIIWAGLPDDVQASLKSKPGVLPELMGCKN

SEQ ID NO: 19 - protein, 245 aa, synthetic construct
  REGION 1..245: note = isolated from library
DTLESIDNCAVGCPTGGSSNVSIVRHAYTLNNNSTTKFANWVAYHITKDTPASGKTRNWKTDPALNPADTLAPRDYTGANAALKVDRGHQAPLASLAGVSDWESLNYLSNITPQKSDLNQGAWARLEDQERKLIDRADISSVYTVTGPLYERDMGKLPGTQKAHTIPSAYWKVIFINNSPAVNHYAAFLFDQNTPKGADFCQFRVTVDEIEKRTGLIIWAGLPDDVQASLKSKPGVLPELMGCKN

SEQ ID NO: 20 - protein, 245 aa, synthetic construct
  REGION 1..245: note = isolated from library
DTLESIDNCAVGCPTGGSSNVSIVRHAYTLNNNSTTKFANWVAYHITKDTPASGKTRNWKTDPALNPADTLAPKDYTGANAALKVDRGHQAPLASLAGVSDWESLNYLSNITPQKSDLNQGAWARLEDQERKLIDRADISSVYTVTGPLYERDMGKLPGTQKAHTIPSAYWKVIFINNSPAVNHYAAFLFDQNTPKGADFCQFRVTVDEIEKRTGLIIWAGLPDDVQASLKSKPGVLPELMGCKN

SEQ ID NO: 21 - protein, 245 aa, synthetic construct
  REGION 1..245: note = isolated from library
DTLESIDNCAVGCPTGGSSNVSIVRHAYTLNNNSTTKFANWVAYHITKDTPASGKTRNWKTDPALNPADTLAPADYLGANAALKVDRGHQAPLASLAGVSDWESLNYLSNITPQKSDLNQGAWARLEDQERKLIDRADISSVYTVTGPLYERDMGKLPGTQKAHTIPSAYWKVIFINNSPAVNHYAAFLFDQNTPKGADFCQFRVTVDEIEKRTGLIIWAGLPDDVQASLKSKPGVLPELMGCKN

SEQ ID NO: 22 - protein, 245 aa, synthetic construct
  REGION 1..245: note = isolated from library
DTLESIDNCAVGCPTGGSSNVSIVRHAYTLNNNSTTKFANWVAYHITKDTPASGKTRNWKTDPALNPADTLAPADYKGANAALKVDRGHQAPLASLAGVSDWESLNYLSNITPQKSDLNQGAWARLEDQERKLIDRADISSVYTVTGPLYERDMGKLPGTQKAHTIPSAYWKVIFINNSPAVNHYAAFLFDQNTPKGADFCQFRVTVDEIEKRTGLIIWAGLPDDVQASLKSKPGVLPELMGCKN

SEQ ID NO: 23 - protein, 245 aa, synthetic construct
  REGION 1..245: note = isolated from library
DTLESIDNCAVGCPTGGSSNVSIVRHAYTLNNNSTTKFANWVAYHITKDTPASGKTRNWKTDPALNPADTLAPADYFGANAALKVDRGHQAPLASLAGVSDWESLNYLSNITPQKSDLNQGAWARLEDQERKLIDRADISSVYTVTGPLYERDMGKLPGTQKAHTIPSAYWKVIFINNSPAVNHYAAFLFDQNTPKGADFCQFRVTVDEIEKRTGLIIWAGLPDDVQASLKSKPGVLPELMGCKN

SEQ ID NO: 24 - protein, 245 aa, synthetic construct
  REGION 1..245: note = isolated from library
DTLESIDNCAVGCPTGGSSNVSIVRHAYTLNNNSTTKFANWVAYHITKDTPASGKTRNWKTDPALNPADTLAPADYRGANAALKVDRGHQAPLASLAGVSDWESLNYLSNITPQKSDLNQGAWARLEDQERKLIDRADISSVYTVTGPLYERDMGKLPGTQKAHTIPSAYWKVIFINNSPAVNHYAAFLFDQNTPKGADFCQFRVTVDEIEKRTGLIIWAGLPDDVQASLKSKPGVLPELMGCKN

SEQ ID NO: 25 - protein, 245 aa, synthetic construct
  REGION 1..245: note = isolated from library
DTLESIDNCAVGCPTGGSSNVSIVRHAYTLNNNSTTKFANWVAYHITKDTPASGKTRNWKTDPALNPADTLAPADYTGAHAALKVDRGHQAPLASLAGVSDWESLNYLSNITPQKSDLNQGAWARLEDQERKLIDRADISSVYTVTGPLYERDMGKLPGTQKAHTIPSAYWKVIFINNSPAVNHYAAFLFDQNTPKGADFCQFRVTVDEIEKRTGLIIWAGLPDDVQASLKSKPGVLPELMGCKN

SEQ ID NO: 26 - protein, 245 aa, synthetic construct
  REGION 1..245: note = isolated from library
DTLESIDNCAVGCPTGGSSNVSIVRHAYTLNNNSTTKFANWVAYHITKDTPASGKTRNWKTDPALNPADTLAPADYTGANAALGVDRGHQAPLASLAGVSDWESLNYLSNITPQKSDLNQGAWARLEDQERKLIDRADISSVYTVTGPLYERDMGKLPGTQKAHTIPSAYWKVIFINNSPAVNHYAAFLFDQNTPKGADFCQFRVTVDEIEKRTGLIIWAGLPDDVQASLKSKPGVLPELMGCKN

SEQ ID NO: 27 - protein, 245 aa, synthetic construct
  REGION 1..245: note = isolated from library
DTLESIDNCAVGCPTGGSSNVSIVRHAYTLNNNSTTKFANWVAYHITKDTPASGKTRNWKTDPALNPADTLAPADYTGANAALKVSRGHQAPLASLAGVSDWESLNYLSNITPQKSDLNQGAWARLEDQERKLIDRADISSVYTVTGPLYERDMGKLPGTQKAHTIPSAYWKVIFINNSPAVNHYAAFLFDQNTPKGADFCQFRVTVDEIEKRTGLIIWAGLPDDVQASLKSKPGVLPELMGCKN

SEQ ID NO: 28 - protein, 245 aa, synthetic construct
  REGION 1..245: note = isolated from library
DTLESIDNCAVGCPTGGSSNVSIVRHAYTLNNNSTTKFANWVAYHITKDTPASGKTRNWKTDPALNPADTLAPADYTGANAALKVDRGHQAPLASLAGVSDWESLNYLSNITPQKKDLNQGAWARLEDQERKLIDRADISSVYTVTGPLYERDMGKLPGTQKAHTIPSAYWKVIFINNSPAVNHYAAFLFDQNTPKGADFCQFRVTVDEIEKRTGLIIWAGLPDDVQASLKSKPGVLPELMGCKN

SEQ ID NO: 29 - protein, 245 aa, synthetic construct
  REGION 1..245: note = isolated from library
DTLESIDNCAVGCPTGGSSNVSIVRHAYTLNNNSTTKFANWVAYHITKDTPASGKTRNWKTDPALNPADTLAPADYTGANAALKVDRGHQAPLASLAGVSDWESLNYLSNITPQKSKLNQGAWARLEDQERKLIDRADISSVYTVTGPLYERDMGKLPGTQKAHTIPSAYWKVIFINNSPAVNHYAAFLFDQNTPKGADFCQFRVTVDEIEKRTGLIIWAGLPDDVQASLKSKPGVLPELMGCKN

SEQ ID NO: 30 - protein, 245 aa, synthetic construct
  REGION 1..245: note = isolated from library
DTLESIDNCAVGCPTGGSSNVSIVRHAYTLNNNSTTKFANWVAYHITKDTPASGKTRNWKTDPALNPADTLAPADYTGANAALKVDRGHQAPLASLAGVSDWESLNYLSNITPQKSALNQGAWARLEDQERKLIDRADISSVYTVTGPLYERDMGKLPGTQKAHTIPSAYWKVIFINNSPAVNHYAAFLFDQNTPKGADFCQFRVTVDEIEKRTGLIIWAGLPDDVQASLKSKPGVLPELMGCKN

SEQ ID NO: 31 - protein, 245 aa, synthetic construct
  REGION 1..245: note = isolated from library
DTLESIDNCAVGCPTGGSSNVSIVRHAYTLNNNSTTKFANWVAYHITKDTPASGKTRNWKTDPALNPADTLAPADYTGANAALKVDRGHQAPLASLAGVSDWESLNYLSNITPQKSSLNQGAWARLEDQERKLIDRADISSVYTVTGPLYERDMGKLPGTQKAHTIPSAYWKVIFINNSPAVNHYAAFLFDQNTPKGADFCQFRVTVDEIEKRTGLIIWAGLPDDVQASLKSKPGVLPELMGCKN

SEQ ID NO: 32 - protein, 245 aa, synthetic construct
  REGION 1..245: note = isolated from library
DTLESIDNCAVGCPTGGSSNVSIVRHAYTLNNNSTTKFANWVAYHITKDTPASGKTRNWKTDPALNPADTLAPADYTGANAALKVDRGHQAPLASLAGVSDWESLNYLSNITPQKSNLNQGAWARLEDQERKLIDRADISSVYTVTGPLYERDMGKLPGTQKAHTIPSAYWKVIFINNSPAVNHYAAFLFDQNTPKGADFCQFRVTVDEIEKRTGLIIWAGLPDDVQASLKSKPGVLPELMGCKN

SEQ ID NO: 33 - protein, 245 aa, synthetic construct
  REGION 1..245: note = isolated from library
DTLESIDNCAVGCPTGGSSNVSIVRHAYTLNNNSTTKFANWVAYHITKDTPASGKTRNWKTDPALNPADTLAPADYTGANAALKVDRGHQAPLASLAGVSDWESLNYLSNITPQKSRLNQGAWARLEDQERKLIDRADISSVYTVTGPLYERDMGKLPGTQKAHTIPSAYWKVIFINNSPAVNHYAAFLFDQNTPKGADFCQFRVTVDEIEKRTGLIIWAGLPDDVQASLKSKPGVLPELMGCKN

SEQ ID NO: 34 - protein, 245 aa, synthetic construct
  REGION 1..245: note = isolated from library
DTLESIDNCAVGCPTGGSSNVSIVRHAYTLNNNSTTKFANWVAYHITKDTPASGKTRNWKTDPALNPADTLAPADYTGANAALKVDRGHQAPLASLAGVSDWESLNYLSNITPQKSDLNQGAWKRLEDQERKLIDRADISSVYTVTGPLYERDMGKLPGTQKAHTIPSAYWKVIFINNSPAVNHYAAFLFDQNTPKGADFCQFRVTVDEIEKRTGLIIWAGLPDDVQASLKSKPGVLPELMGCKN

SEQ ID NO: 35 - protein, 245 aa, synthetic construct
  REGION 1..245: note = isolated from library
DTLESIDNCAVGCPTGGSSNVSIVRHAYTLNNNSTTKFANWVAYHITKDTPASGKTRNWKTDPALNPADTLAPADYTGANAALKVDRGHQAPLASLAGVSDWESLNYLSNITPQKSDLNQGAWRRLEDQERKLIDRADISSVYTVTGPLYERDMGKLPGTQKAHTIPSAYWKVIFINNSPAVNHYAAFLFDQNTPKGADFCQFRVTVDEIEKRTGLIIWAGLPDDVQASLKSKPGVLPELMGCKN

SEQ ID NO: 36 - protein, 245 aa, synthetic construct
  REGION 1..245: note = isolated from library
DTLESIDNCAVGCPTGGSSNVSIVRHAYTLNNNSTTKFANWVAYHITKDTPASGKTRNWKTDPALNPADTLAPADYTGANAALKVDRGHQAPLASLAGVSDWESLNYLSNITPQKSDLNQGAWARLEMQERKLIDRADISSVYTVTGPLYERDMGKLPGTQKAHTIPSAYWKVIFINNSPAVNHYAAFLFDQNTPKGADFCQFRVTVDEIEKRTGLIIWAGLPDDVQASLKSKPGVLPELMGCKN

SEQ ID NO: 37 - protein, 245 aa, synthetic construct
  REGION 1..245: note = isolated from library
DTLESIDNCAVGCPTGGSSNVSIVRHAYTLNNNSTTKFANWVAYHITKDTPASGKTRNWKTDPALNPADTLAPADYTGANAALKVDRGHQAPLASLAGVSDWESLNYLSNITPQKSDLNQGAWARLEYQERKLIDRADISSVYTVTGPLYERDMGKLPGTQKAHTIPSAYWKVIFINNSPAVNHYAAFLFDQNTPKGADFCQFRVTVDEIEKRTGLIIWAGLPDDVQASLKSKPGVLPELMGCKN

SEQ ID NO: 38 - protein, 245 aa, synthetic construct
  REGION 1..245: note = isolated from library
DTLESIDNCAVGCPTGGSSNVSIVRHAYTLNNNSTTKFANWVAYHITKDTPASGKTRNWKTDPALNPADTLAPADYTGANAALKVDRGHQAPLASLAGVSDWESLNYLSNITPQKSDLNQGAWARLEKQERKLIDRADISSVYTVTGPLYERDMGKLPGTQKAHTIPSAYWKVIFINNSPAVNHYAAFLFDQNTPKGADFCQFRVTVDEIEKRTGLIIWAGLPDDVQASLKSKPGVLPELMGCKN

SEQ ID NO: 39 - protein, 245 aa, synthetic construct
  REGION 1..245: note = isolated from library
DTLESIDNCAVGCPTGGSSNVSIVRHAYTLNNNSTTKFANWVAYHITKDTPASGKTRNWKTDPALNPADTLAPADYTGANAALKVDRGHQAPLASLAGVSDWESLNYLSNITPQKSDLNQGAWARLESQERKLIDRADISSVYTVTGPLYERDMGKLPGTQKAHTIPSAYWKVIFINNSPAVNHYAAFLFDQNTPKGADFCQFRVTVDEIEKRTGLIIWAGLPDDVQASLKSKPGVLPELMGCKN

SEQ ID NO: 40 - protein, 245 aa, synthetic construct
  REGION 1..245: note = isolated from library
DTLESIDNCAVGCPTGGSSNVSIVRHAYTLNNNSTTKFANWVAYHITKDTPASGKTRNWKTDPALNPADTLAPADYTGANAALKVDRGHQAPLASLAGVSDWESLNYLSNITPQKSDLNQGAWARLENQERKLIDRADISSVYTVTGPLYERDMGKLPGTQKAHTIPSAYWKVIFINNSPAVNHYAAFLFDQNTPKGADFCQFRVTVDEIEKRTGLIIWAGLPDDVQASLKSKPGVLPELMGCKN

SEQ ID NO: 41 - protein, 245 aa, synthetic construct
  REGION 1..245: note = isolated from library
DTLESIDNCAVGCPTGGSSNVSIVRHAYTLNNNSTTKFANWVAYHITKDTPASGKTRNWKTDPALNPADTLAPADYTGANAALKVDRGHQAPLASLAGVSDWESLNYLSNITPQKSDLNQGAWARLEFQERKLIDRADISSVYTVTGPLYERDMGKLPGTQKAHTIPSAYWKVIFINNSPAVNHYAAFLFDQNTPKGADFCQFRVTVDEIEKRTGLIIWAGLPDDVQASLKSKPGVLPELMGCKN

SEQ ID NO: 42 - protein, 245 aa, synthetic construct
  REGION 1..245: note = isolated from library
DTLESIDNCAVGCPTGGSSNVSIVRHAYTLNNNSTTKFANWVAYHITKDTPASGKTRNWKTDPALNPADTLAPADYTGANAALKVDRGHQAPLASLAGVSDWESLNYLSNITPQKSDLNQGAWARLEGQERKLIDRADISSVYTVTGPLYERDMGKLPGTQKAHTIPSAYWKVIFINNSPAVNHYAAFLFDQNTPKGADFCQFRVTVDEIEKRTGLIIWAGLPDDVQASLKSKPGVLPELMGCKN

SEQ ID NO: 43 - protein, 245 aa, synthetic construct
  REGION 1..245: note = isolated from library
DTLESIDNCAVGCPTGGSSNVSIVRHAYTLNNNSTTKFANWVAYHITKDTPASGKTRNWKTDPALNPADTLAPADYTGANAALKVDRGHQAPLASLAGVSDWESLNYLSNITPQKSDLNQGAWARLERQERKLIDRADISSVYTVTGPLYERDMGKLPGTQKAHTIPSAYWKVIFINNSPAVNHYAAFLFDQNTPKGADFCQFRVTVDEIEKRTGLIIWAGLPDDVQASLKSKPGVLPELMGCKN

SEQ ID NO: 44 - protein, 245 aa, synthetic construct
  REGION 1..245: note = isolated from library
DTLESIDNCAVGCPTGGSSNVSIVRHAYTLNNNSTTKFANWVAYHITKDTPASGKTRNWKTDPALNPADTLAPADYTGANAALKVDRGHQAPLASLAGVSDWESLNYLSNITPQKSDLNQGAWARLEDQERKLINRADISSVYTVTGPLYERDMGKLPGTQKAHTIPSAYWKVIFINNSPAVNHYAAFLFDQNTPKGADFCQFRVTVDEIEKRTGLIIWAGLPDDVQASLKSKPGVLPELMGCKN

SEQ ID NO: 45 - protein, 245 aa, synthetic construct
  REGION 1..245: note = isolated from library
DTLESIDNCAVGCPTGGSSNVSIVRHAYTLNNNSTTKFANWVAYHITKDTPASGKTRNWKTDPALNPADTLAPADYTGANAALKVDRGHQAPLASLAGVSDWESLNYLSNITPQKSDLNQGAWARLEDQERKLIKRADISSVYTVTGPLYERDMGKLPGTQKAHTIPSAYWKVIFINNSPAVNHYAAFLFDQNTPKGADFCQFRVTVDEIEKRTGLIIWAGLPDDVQASLKSKPGVLPELMGCKN

SEQ ID NO: 46 - protein, 245 aa, synthetic construct
  REGION 1..245: note = isolated from library
DTLESIDNCAVGCPTGGSSNVSIVRHAYTLNNNSTTKFANWVAYHITKDTPASGKTRNWKTDPALNPADTLAPADYTGANAALKVDRGHQAPLASLAGVSDWESLNYLSNITPQKSDLNQGAWARLEDQERKLIGRADISSVYTVTGPLYERDMGKLPGTQKAHTIPSAYWKVIFINNSPAVNHYAAFLFDQNTPKGADFCQFRVTVDEIEKRTGLIIWAGLPDDVQASLKSKPGVLPELMGCKN

SEQ ID NO: 47 - protein, 245 aa, synthetic construct
  REGION 1..245: note = isolated from library
DTLESIDNCAVGCPTGGSSNVSIVRHAYTLNNNSTTKFANWVAYHITKDTPASGKTRNWKTDPALNPADTLAPADYTGANAALKVDRGHQAPLASLAGVSDWESLNYLSNITPQKSDLNQGAWARLEDQERKLIRRADISSVYTVTGPLYERDMGKLPGTQKAHTIPSAYWKVIFINNSPAVNHYAAFLFDQNTPKGADFCQFRVTVDEIEKRTGLIIWAGLPDDVQASLKSKPGVLPELMGCKN

SEQ ID NO: 48 - protein, 245 aa, synthetic construct
  REGION 1..245: note = isolated from library
DTLESIDNCAVGCPTGGSSNVSIVRHAYTLNNNSTTKFANWVAYHITKDTPASGKTRNWKTDPALNPADTLAPADYTGANAALKVDRGHQAPLASLAGVSDWESLNYLSNITPQKSDLNQGAWARLEDQERKLIDRADISSVYTVTGPLYERDMGKLPGTQKAHTIPSAYWKVIFINNSPAVNHYAAFLFPQNTPKGADFCQFRVTVDEIEKRTGLIIWAGLPDDVQASLKSKPGVLPELMGCKN

SEQ ID NO: 49 - protein, 245 aa, synthetic construct
  REGION 1..245: note = isolated from library
DTLESIDNCAVGCPTGGSSNVSIVRHAYTLNNNSTTKFANWVAYHITKDTPASGKTRNWKTDPALNPADTLAPADYTGANAALKVDRGHQAPLASLAGVSDWESLNYLSNITPQKSDLNQGAWARLEDQERKLIDRADISSVYTVTGPLYERDMGKLPGTQKAHTIPSAYWKVIFINNSPAVNHYAAFLFDQNTPKKADFCQFRVTVDEIEKRTGLIIWAGLPDDVQASLKSKPGVLPELMGCKN

SEQ ID NO: 50 - protein, 245 aa, synthetic construct
  REGION 1..245: note = isolated from library
DTLESIDNCAVGCPTGGSSNVSIVRHAYTLNNNSTTKFANWVAYHITKDTPASGKTRNWKTDPALNPADTLAPADYTGANAALKVDRGHQAPLASLAGVSDWESLNYLSNITPQKSDLNQGAWARLEDQERKLIDRADISSVYTVTGPLYERDMGKLPGTQKAHTIPSAYWKVIFINNSPAVNHYAAFLFDQNTPKGANFCQFRVTVDEIEKRTGLIIWAGLPDDVQASLKSKPGVLPELMGCKN

SEQ ID NO: 51 - protein, 245 aa, synthetic construct
  REGION 1..245: note = isolated from library
DTLESIDNCAVGCPTGGSSNVSIVRHAYTLNNNSTTKFANWVAYHITKDTPASGKTRNWKTDPALNPADTLAPADYTGANAALKVDRGHQAPLASLAGVSDWESLNYLSNITPQKSDLNQGAWARLEDQERKLIDRADISSVYTVTGPLYERDMGKLPGTQKAHTIPSAYWKVIFINNSPAVNHYAAFLFDQNTPKGAKFCQFRVTVDEIEKRTGLIIWAGLPDDVQASLKSKPGVLPELMGCKN

SEQ ID NO: 52 - protein, 245 aa, synthetic construct
  REGION 1..245: note = isolated from library
DTLESIDNCAVGCPTGGSSNVSIVRHAYTLNNNSTTKFANWVAYHITKDTPASGKTRNWKTDPALNPADTLAPADYTGANAALKVDRGHQAPLASLAGVSDWESLNYLSNITPQKSDLNQGAWARLEDQERKLIDRADISSVYTVTGPLYERDMGKLPGTQKAHTIPSAYWKVIFINNSPAVNHYAAFLFDQNTPKGASFCQFRVTVDEIEKRTGLIIWAGLPDDVQASLKSKPGVLPELMGCKN

SEQ ID NO: 53 - protein, 245 aa, synthetic construct
  REGION 1..245: note = isolated from library
DTLESIDNCAVGCPTGGSSNVSIVRHAYTLNNNSTTKFANWVAYHITKDTPASGKTRNWKTDPALNPADTLAPADYTGANAALKVDRGHQAPLASLAGVSDWESLNYLSNITPQKSDLNQGAWARLEDQERKLIDRADISSVYTVTGPLYERDMGKLPGTQKAHTIPSAYWKVIFINNSPAVNHYAAFLFDQNTPKGADFCQFQVTVDEIEKRTGLIIWAGLPDDVQASLKSKPGVLPELMGCKN

SEQ ID NO: 54 - protein, 245 aa, synthetic construct
  REGION 1..245: note = isolated from library
DTLESIDNCAVGCPTGGSSNVSIVRHAYTLNNNSTTKFANWVAYHITKDTPASGKTRNWKTDPALNPADTLAPADYTGANAALKVDRGHQAPLASLAGVSDWESLNYLSNITPQKSDLNQGAWARLEDQERKLIDRADISSVYTVTGPLYERDMGKLPGTQKAHTIPSAYWKVIFINNSPAVNHYAAFLFDQNTPKGADFCQFRVTVDEIEKRTGLIIWAGLPDDVQASLKSKPGVLPALMGCKN

SEQ ID NO: 55 - protein, 245 aa, synthetic construct
  REGION 1..245: note = isolated from library
DTLESIDNCAVGCPTGGSSNVSIVRHAYTLNNNSTTKFANWVAYHITKDTLASGKTRRWKTDPALNPADTLAPADYKGANAALKVDRGHQAPLASLAGVSDWESLNYLSNITPQKSDLNQGAWKRLEDQERKLIDRADISSVYTVTGPLYERDMGKLPGTQKAHTIPSAYWKVIFINNSPAVNHYAAFLFDQNTPKKADFCQFRVTVDEIEKRTGLIIWAGLPDDVQASLKSKPGVLPELMGCKN

SEQ ID NO: 56 - protein, 245 aa, synthetic construct
  REGION 1..245: note = isolated from library
DTLESIDNCAVGCPTGGSSNVSIVRHAYTLNNNSTTKFANWVAYHITKDTPASGKTRRWKTDPALNPADTLAPADYRGANAALKVDRGHQAPLASLAGVSDWESLNYLSNITPQKSDLNQGAWKRLEDQERKLIDRADISSVYTVTGPLYERDMGKLPGTQKAHTIPSAYWKVIFINNSPAVNHYAAFLFDQNTPKKADFCQFRVTVDEIEKRTGLIIWAGLPDDVQASLKSKPGVLPELMGCKN

SEQ ID NO: 57 - protein, 245 aa, synthetic construct
  REGION 1..245: note = isolated from library
DTLESIDNCAVGCPTGGSSNVSIVRHAYTLNNNSTTKFANWVAYHITKDTLASGKTRRWKTDPALNPADTLAPADYKGANAALKVDRGHQAPLASLAGVSDWESLNYLSNITPQKSDLNQGAWKRLEDQERKLIDRADISSVYTVTGPLYERDMGKLPGTQKAHTIPSAYWKVIFINNSPAVNHYAAFLFDQNTPKGADFCQFRVTVDEIEKRTGLIIWAGLPDDVQASLKSKPGVLPELMGCKN

SEQ ID NO: 58 - protein, 245 aa, synthetic construct
  REGION 1..245: note = isolated from library
DTLESIDNCAVGCPTGGSSNVSIVRHAYTLNNNSTTKFANWVAYHITKDTLASGKRRNWKTDPALNPADTLAPADYKGANAALKVDRGHQAPLASLAGVSDWESLNYLSNITPQKSDLNQGAWKRLEDQERKLIDRADISSVYTVTGPLYERDMGKLPGTQKAHTIPSAYWKVIFINNSPAVNHYAAFLFDQNTPKKADFCQFRVTVDEIEKRTGLIIWAGLPDDVQASLKSKPGVLPELMGCKN

SEQ ID NO: 59 - protein, 245 aa, synthetic construct
  REGION 1..245: note = isolated from library
DTLESIDNCAVGCPTGGSSNVSIVRHAYTLNNNSTTKFANWVAYHITKDTLASGKTRNWKTDPALNPADTLAPADYRGANAALKVDRGHQAPLASLAGVSDWESLNYLSNITPQKSDLNQGAWKRLEDQERKLIDRADISSVYTVTGPLYERDMGKLPGTQKAHTIPSAYWKVIFINNSPAVNHYAAFLFDQNTPKKADFCQFRVTVDEIEKRTGLIIWAGLPDDVQASLKSKPGVLPELMGCKN

SEQ ID NO: 60 - protein, 245 aa, synthetic construct
  REGION 1..245: note = isolated from library
DTLESIDNCAVGCPTGGSSNVSIVRHAYTLNNNSTTKFANWVAYHITKDTLASGKTRRWKTDPALNPADTLAPADYTGANAALKVDRGHQAPLASLAGVSDWESLNYLSNITPQKSDLNQGAWKRLEDQERKLIDRADISSVYTVTGPLYERDMGKLPGTQKAHTIPSAYWKVIFINNSPAVNHYAAFLFDQNTPKKADFCQFRVTVDEIEKRTGLIIWAGLPDDVQASLKSKPGVLPELMGCKN

SEQ ID NO: 61 - protein, 245 aa, synthetic construct
  REGION 1..245: note = isolated from library
DTLESIDNCAVGCPTGGSSNVSIVRHAYTLNNNSTTKFANWVAYHITKDTLASGKRRNWKTDPALNPADTLAPADYRGANAALKVDRGHQAPLASLAGVSDWESLNYLSNITPQKSDLNQGAWKRLEDQERKLIDRADISSVYTVTGPLYERDMGKLPGTQKAHTIPSAYWKVIFINNSPAVNHYAAFLFDQNTPKGADFCQFRVTVDEIEKRTGLIIWAGLPDDVQASLKSKPGVLPELMGCKN

SEQ ID NO: 62 - protein, 245 aa, synthetic construct
  REGION 1..245: note = isolated from library
DTLESIDNCAVGCPTGGSSNVSIVRHAYTLNNNSTTKFANWVAYHITKDTPASGKRRNWKTDPALNPADTLAPADYKGANAALKVDRGHQAPLASLAGVSDWESLNYLSNITPQKSDLNQGAWKRLEDQERKLIDRADISSVYTVTGPLYERDMGKLPGTQKAHTIPSAYWKVIFINNSPAVNHYAAFLFDQNTPKGADFCQFRVTVDEIEKRTGLIIWAGLPDDVQASLKSKPGVLPELMGCKN

SEQ ID NO: 63 - protein, 245 aa, synthetic construct
  REGION 1..245: note = isolated from library
DTLESIDNCAVGCPTGGSSNVSIVRHAYTLNNNSTTKFANWVAYHITKDTLASGKRRRWKTDPALNPADTLAPADYTGANAALKVDRGHQAPLASLAGVSDWESLNYLSNITPQKSDLNQGAWKRLEDQERKLIDRADISSVYTVTGPLYERDMGKLPGTQKAHTIPSAYWKVIFINNSPAVNHYAAFLFDQNTPKGADFCQFRVTVDEIEKRTGLIIWAGLPDDVQASLKSKPGVLPELMGCKN

SEQ ID NO: 64 - protein, 245 aa, synthetic construct
  REGION 1..245: note = isolated from library
DTLESIDNCAVGCPTGGSSNVSIVRHAYTLNNNSTTKFANWVAYHITKDTLASGKTRNWKTDPALNPADTLAPADYRGANAALKVDRGHQAPLASLAGVSDWESLNYLSNITPQKSDLNQGAWKRLEDQERKLIDRADISSVYTVTGPLYERDMGKLPGTQKAHTIPSAYWKVIFINNSPAVNHYAAFLFDQNTPKGADFCQFRVTVDEIEKRTGLIIWAGLPDDVQASLKSKPGVLPELMGCKN

SEQ ID NO: 65 - protein, 245 aa, synthetic construct
  REGION 1..245: note = isolated from library
DTLESIDNCAVGCPTGGSSNVSIVRHAYTLNNNSTTKFANWVAYHITKDTLASGKTRRWKTDPALNPADTLAPADYTGANAALKVDRGHQAPLASLAGVSDWESLNYLSNITPQKSDLNQGAWKRLEDQERKLIDRADISSVYTVTGPLYERDMGKLPGTQKAHTIPSAYWKVIFINNSPAVNHYAAFLFDQNTPKGADFCQFRVTVDEIEKRTGLIIWAGLPDDVQASLKSKPGVLPELMGCKN

SEQ ID NO: 66 - protein, 245 aa, synthetic construct
  REGION 1..245: note = isolated from library
DTLESIDNCAVGCPTGGSSNVSIVRHAYTLNNNSTTKFANWVAYHITKDTLASGKTRRWKTDPALNPADTLAPADYRGANAALKVDRGHQAPLASLAGVSDWESLNYLSNITPQKSDLNQGAWARLEDQERKLIDRADISSVYTVTGPLYERDMGKLPGTQKAHTIPSAYWKVIFINNSPAVNHYAAFLFDQNTPKGADFCQFRVTVDEIEKRTGLIIWAGLPDDVQASLKSKPGVLPELMGCKN

SEQ ID NO: 67 - protein, 245 aa, synthetic construct
  REGION 1..245: note = isolated from library
DTLESIDNCAVGCPTGGSSNVSIVRHAYTLNNNSTTKFANWVAYHITKDTPASGKTRNWKTDPALNPADTLAPADYKGANAALKVDRGHQAPLASLAGVSDWESLNYLSNITPQKSDLNQGAWKRLEDQERKLIDRADISSVYTVTGPLYERDMGKLPGTQKAHTIPSAYWKVIFINNSPAVNHYAAFLFDQNTPKGADFCQFRVTVDEIEKRTGLIIWAGLPDDVQASLKSKPGVLPELMGCKN

SEQ ID NO: 68 - protein, 245 aa, synthetic construct
  REGION 1..245: note = isolated from library
DTLESIDNCAVGCPTGGSSNVSIVRHAYTLNNNSTTKFANWVAYHITKDTPASGKRRNWKTDPALNPADTLAPADYKGANAALKVDRGHQAPLASLAGVSDWESLNYLSNITPQKSDLNQGAWKRLEDQERKLIRRADISSVYTVTGPLYERDMGKLPGTQKAHTIPSAYWKVIFINNSPAVNHYAAFLFDQNTPKKADFCQFRVTVDEIEKRTGLIIWAGLPDDVQASLKSKPGVLPELMGCKN

SEQ ID NO: 69 - protein, 245 aa, synthetic construct
  REGION 1..245: note = isolated from library
DTLESIDNCAVGCPTGGSSNVSIVRHAYTLNNNSTTKFANWVAYHITKDTLASGKRRRWKTDPALNPADTLAPADYKGANAALKVDRGHQAPLASLAGVSDWESLNYLSNITPQKSDLNQGAWKRLEDQERKLIRRADISSVYTVTGPLYERDMGKLPGTQKAHTIPSAYWKVIFINNSPAVNHYAAFLFDQNTPKGADFCQFRVTVDEIEKRTGLIIWAGLPDDVQASLKSKPGVLPELMGCKN

SEQ ID NO: 70 - protein, 245 aa, synthetic construct
  REGION 1..245: note = isolated from library
DTLESIDNCAVGCPTGGSSNVSIVRHAYTLNNNSTTKFANWVAYHITKDTLASGKTRNWKTDPALNPADTLAPADYTGANAALKVDRGHQAPLASLAGVSDWESLNYLSNITPQKSDLNQGAWKRLERQERKLIRRADISSVYTVTGPLYERDMGKLPGTQKAHTIPSAYWKVIFINNSPAVNHYAAFLFDQNTPKGADFCQFRVTVDEIEKRTGLIIWAGLPDDVQASLKSKPGVLPELMGCKN

SEQ ID NO: 71 - protein, 245 aa, synthetic construct
  REGION 1..245: note = isolated from library
DTLESIDNCAVGCPTGGSSNVSIVRHAYTLNNNSTTKFANWVAYHITKDTLASGKTRRWKTDPALNPADTLAPADYTGANAALKVDRGHQAPLASLAGVSDWESLNYLSNITPQKSDLNQGAWKRLERQERKLIDRADISSVYTVTGPLYERDMGKLPGTQKAHTIPSAYWKVIFINNSPAVNHYAAFLFDQNTPKKADFCQFRVTVDEIEKRTGLIIWAGLPDDVQASLKSKPGVLPELMGCKN

SEQ ID NO: 72 - protein, 245 aa, synthetic construct
  REGION 1..245: note = isolated from library
DTLESIDNCAVGCPTGGSSNVSIVRHAYTLNNNSTTKFANWVAYHITKDTLASGKTRRWKTDPALNPADTLAPADYTGANAALKVDRGHQAPLASLAGVSDWESLNYLSNITPQKSDLNQGAWKRLERQERKLIRRADISSVYTVTGPLYERDMGKLPGTQKAHTIPSAYWKVIFINNSPAVNHYAAFLFDQNTPKGADFCQFRVTVDEIEKRTGLIIWAGLPDDVQASLKSKPGVLPELMGCKN

SEQ ID NO: 73 - protein, 245 aa, synthetic construct
  REGION 1..245: note = isolated from library
DTLESIDNCAVGCPTGGSSNVSIVRHAYTLNNNSTTKFANWVAYHITKDTLASGKPRNWKTDPALNPADTLAPADYTGANAALKVDRGHQAPLASLAGVSDWESLNYLSNITPQKSDLNQGAWARLEDQERKLINRADISSVYTVTGPLYERDMGKLPGTQKAHTIPSAYWKVIFINNSPAVNHYAAFLFDQNTPKGADFCQFRVTVDEIEKRTGLIIWAGLPDDVQASLKSKPGVLPELMGCKN

SEQ ID NO: 74 - protein, 245 aa, synthetic construct
  REGION 1..245: note = isolated from library
DTLESIDNCAVGCPTGGSSNVSIVRHAYTLNNNSTTKFANWVAYHITKDTLASGKPRNWKTDPALNPADTLAPADYTGANAALKVDRGHQAPLASLAGVSDWESLNYLSNITPQKSDLNQGAWARLEDQERKLIDRADISSVYTVTGPLYERDMGKLPGTQKAHTIPSAYWKVIFINNSPAVNHYAAFLFDQNTPKGADFCQFRVTVDEIEKRTGLIIWAGLPDDVQASLKSKPGVLPELMGCKN

SEQ ID NO: 75 - protein, 245 aa, synthetic construct
  REGION 1..245: note = isolated from library
DTLESIDNCAVGCPTGGSSNVSIVRHAYTLNNNSTTKFANWVAYHITKDTLASGKPRNWKTDPALNPADTLAPADYTGANAALGVDRGHQAPLASLAGVSDWESLNYLSNITPQKSDLNQGAWARLEDQERKLIDRADISSVYTVTGPLYERDMGKLPGTQKAHTIPSAYWKVIFINNSPAVNHYAAFLFDQNTPKGADFCQFRVTVDEIEKRTGLIIWAGLPDDVQASLKSKPGVLPELMGCKN

SEQ ID NO: 76 - protein, 245 aa, synthetic construct
  REGION 1..245: note = isolated from library
DTLESIDNCAVGCPTGGSSNVSIVRHAYTLNNNSTTKFANWVAYHITKDTPASGKPRNWKTDPALNPADTLAPADYTGANAALGVDRGHQAPLASLAGVSDWESLNYLSNITPQKSDLNQGAWARLEDQERKLIDRADISSVYTVTGPLYERDMGKLPGTQKAHTIPSAYWKVIFINNSPAVNHYAAFLFDQNTPKGADFCQFRVTVDEIEKRTGLIIWAGLPDDVQASLKSKPGVLPELMGCKN

SEQ ID NO: 77 - protein, 245 aa, synthetic construct
  REGION 1..245: note = isolated from library
DTLESIDNCAVGCPTGGSSNVSIVRHAYTLNNNSTTKFANWVAYHITKDTLASGKDRNWKTDPALNPADTLAPADYTGANAALKVDRGHQAPLASLAGVSDWESLNYLSNITPQKSDLNQGAWARLEDQERKLIDRADISSVYTVTGPLYERDMGKLPGTQKAHTIPSAYWKVIFINNSPAVNHYAAFLFDQNTPKGADFCQFRVTVDEIEKRTGLIIWAGLPDDVQASLKSKPGVLPELMGCKN

SEQ ID NO: 78 - protein, 245 aa, synthetic construct
  REGION 1..245: note = isolated from library
DTLESIDNCAVGCPTGGSSNVSIVRHAYTLNNNSTTKFANWVAYHITKDTLASGKDRNWKTDPALNPADTLAPADYTGANAALKVDRGHQAPLASLAGVSDWESLNYLSNITPQKSDLNRGAWARLEDQERKLIDRADISSVYTVTGPLYERDMGKLPGTQKAHTIPSAYWKVIFINNSPAVNHYAAFLFDQNTPKGADFCQFRVTVDEIEKRTGLIIWAGLPDDVQASLKSKPGVLPELMGCKN

SEQ ID NO: 79 - protein, 245 aa, synthetic construct
  REGION 1..245: note = isolated from library
DTLESIDNCAVGCPTGGSSNVSIVRHAYTLNNNSTTKFANWVAYHITKDTLASGKKRNWKTDPALNPADTLAPADYTGANAALKVDRGHQAPLASLAGVSDWESLNYLSNITPQKSDLNQGAWARLEDQERKLIDRADISSVYTVTGPLYERDMGKLPGTQKAHTIPSAYWKVIFINNSPAVNHYAAFLFDQNTPKGADFCQFRVTVDEIEKRTGLIIWAGLPDDVQASLKSKPGVLPELMGCKN

SEQ ID NO: 80 - protein, 245 aa, synthetic construct
  REGION 1..245: note = isolated from library
DTLESIDNCAVGCPTGGSSNVSIVRHAYTLNNNSTTKFANWVAYHITKDTLASGKSRNWKTDPALNPADTLAPADYTGANAALKVDRGHQAPLASLAGVSDWESLNYLSNITPQKSDLNQGAWARLEDQERKLIDRADISSVYTVTGPLYERDMGKLPGTQKAHTIPSAYWKVIFINNSPAVNHYAAFLFDQNTPKGADFCQFRVTVDEIEKRTGLIIWAGLPDDVQASLKSKPGVLPELMGCKN

SEQ ID NO: 81 - protein, 245 aa, synthetic construct; identical to SEQ ID NO: 74
  REGION 1..245: note = isolated from library

SEQ ID NO: 82 - protein, 245 aa, synthetic construct
  REGION 1..245: note = isolated from library
DTLESIDNCAVGCPTGGSSNVSIVRHAYTLNNNSTTKFANWVAYHITKDTLASGKDRNWKTDPALNPADTLAPADYTGANAALKVDRGHQAPLASLAGVSDWESLNYLSNITPQKSDLNQGAWARLESQERKLIDRADISSVYTVTGPLYERDMGKLPGTQKAHTIPSAYWKVIFINNSPAVNHYAAFLFDQNTPKGADFCQFRVTVDEIEKRTGLIIWAGLPDDVQASLKSKPGVLPELMGCKN

SEQ ID NO: 83 - protein, 245 aa, synthetic construct
  REGION 1..245: note = isolated from library
DTLESIDNCAVGCPTGGSSNVSIVRHAYTLNNNSTTKFANWVAYHITKDTLASGKGRNWKTDPALNPADTLAPADYTGANAALKVDRGHQAPLASLAGVSDWESLNYLSNITPQKSDLNQGAWARLEDQERKLIDRADISSVYTVTGPLYERDMGKLPGTQKAHTIPSAYWKVIFINNSPAVNHYAAFLFDQNTPKGADFCQFRVTVDEIEKRTGLIIWAGLPDDVQASLKSKPGVLPELMGCKN

SEQ ID NO: 84 - protein, 245 aa, synthetic construct
  REGION 1..245: note = isolated from library
DTLESIDNCAVGCPTGGSSNVSIVRHAYTLNNNSTTKFANWVAYHITKDTLASGKDRNWKTDPALNPADTLAPADYTGANAALKVDRGHQAPLASLAGVSDWESLNYLSNITPQKSDLNQGAWARLENQERKLIDRADISSVYTVTGPLYERDMGKLPGTQKAHTIPSAYWKVIFINNSPAVNHYAAFLFDQNTPKGADFCQFRVTVDEIEKRTGLIIWAGLPDDVQASLKSKPGVLPELMGCKN

SEQ ID NO: 85 - protein, 245 aa, synthetic construct
  REGION 1..245: note = isolated from library
DTLESIDNCAVGCPTGGSSNVSIVRHAYTLNNNSTTKFANWVAYHITKDTLASGKDRNWKTDPALNPADTLAPADYTGANAALKVDRGHQAPLASLAGVSDWESLNYLSNITPQKSRLNQGAWARLEDQERKLIDRADISSVYTVTGPLYERDMGKLPGTQKAHTIPSAYWKVIFINNSPAVNHYAAFLFDQNTPKGADFCQFRVTVDEIEKRTGLIIWAGLPDDVQASLKSKPGVLPELMGCKN

SEQ ID NO: 86 - protein, 245 aa, synthetic construct
  REGION 1..245: note = isolated from library
DTLESIDNCAVGCPTGGSSNVSIVRHAYTLNNNSTTKFANWVAYHITKDTLASGKDRNWKTDPALNPADTLAPADYKGANAALKVDRGHQAPLASLAGVSDWESLNYLSNITPQKSDLNQGAWARLEDQERKLIDRADISSVYTVTGPLYERDMGKLPGTQKAHTIPSAYWKVIFINNSPAVNHYAAFLFDQNTPKGADFCQFRVTVDEIEKRTGLIIWAGLPDDVQASLKSKPGVLPELMGCKN

SEQ ID NO: 87 - protein, 245 aa, synthetic construct
  REGION 1..245: note = isolated from library
DTLESIDNCAVGCPTGGSSNVSIVRHAYTLNNNSTTKFANWVAYHITKDTLASGKDRNWKTDPALNPADTLAPADYTGANAALKVDRGHQAPLASLAGVSDWESLNYLSNITPQKSDLNQGAWARLEGQERKLIDRADISSVYTVTGPLYERDMGKLPGTQKAHTIPSAYWKVIFINNSPAVNHYAAFLFDQNTPKGADFCQFRVTVDEIEKRTGLIIWAGLPDDVQASLKSKPGVLPELMGCKN

SEQ ID NO: 88 - protein, 245 aa, synthetic construct
  REGION 1..245: note = isolated from library
DTLESIDNCAVGCPTGGSSNVSIVRHAYTLNNNSTTKFANWVAYHITKDTLASGKARNWKTDPALNPADTLAPADYTGANAALKVDRGHQAPLASLAGVSDWESLNYLSNITPQKSDLNQGAWARLEDQERKLIDRADISSVYTVTGPLYERDMGKLPGTQKAHTIPSAYWKVIFINNSPAVNHYAAFLFDQNTPKGADFCQFRVTVDEIEKRTGLIIWAGLPDDVQASLKSKPGVLPELMGCKN

SEQ ID NO: 89 - protein, 245 aa, synthetic construct
  REGION 1..245: note = isolated from library
DTLESIDNCAVGCPTGGSSNVSIVRHAYTLNNNSTTKFANWVAYHITKDTLASGKVRNWKTDPALNPADTLAPADYTGANAALKVDRGHQAPLASLAGVSDWESLNYLSNITPQKSDLNQGAWARLEDQERKLIDRADISSVYTVTGPLYERDMGKLPGTQKAHTIPSAYWKVIFINNSPAVNHYAAFLFDQNTPKGADFCQFRVTVDEIEKRTGLIIWAGLPDDVQASLKSKPGVLPELMGCKN

SEQ ID NO: 90 - protein, 245 aa, synthetic construct
  REGION 1..245: note = isolated from library
DTLESIDNCAVGCPTGGSSNVSIVRHAYTLNNNSTTKFANWVAYHITKDTLASGKIRNWKTDPALNPADTLAPADYTGANAALKVDRGHQAPLASLAGVSDWESLNYLSNITPQKSDLNQGAWARLEDQERKLIDRADISSVYTVTGPLYERDMGKLPGTQKAHTIPSAYWKVIFINNSPAVNHYAAFLFDQNTPKGADFCQFRVTVDEIEKRTGLIIWAGLPDDVQASLKSKPGVLPELMGCKN

SEQ ID NO: 91 - protein, 245 aa, synthetic construct
  REGION 1..245: note = isolated from library
DTLESIDNCAVGCPTGGSSNVSIVRHAYTLNNNSTTKFANWVAYHITKDTLASGKDRNWKTDPALNPADTLAPADYTGANAALKVDRGHQAPLASLAGVSDWESLNYLSNITPQKSDLNQGAWARLEDRERKLIDRADISSVYTVTGPLYERDMGKLPGTQKAHTIPSAYWKVIFINNSPAVNHYAAFLFDQNTPKGADFCQFRVTVDEIEKRTGLIIWAGLPDDVQASLKSKPGVLPELMGCKN

SEQ ID NO: 92 - protein, 245 aa, synthetic construct
  REGION 1..245: note = isolated from library
DTLESIDNCAVGCPTGGSSNVSIVRHAYTLNNNSTTKFANWVAYHITKDTLASGKFRNWKTDPALNPADTLAPADYTGANAALKVDRGHQAPLASLAGVSDWESLNYLSNITPQKSDLNQGAWARLEDQERKLIDRADISSVYTVTGPLYERDMGKLPGTQKAHTIPSAYWKVIFINNSPAVNHYAAFLFDQNTPKGADFCQFRVTVDEIEKRTGLIIWAGLPDDVQASLKSKPGVLPELMGCKN

SEQ ID NO: 93 - protein, 245 aa, synthetic construct
  REGION 1..245: note = isolated from library
DTLESIDNCAVGCPTGGSSNVSIVRHAYTLNNNSTTKFANWVAYHITKDTLASGKDRNWKTDPALNPADTLAPADYTGANAALKVDRGHQAPLASLAGVSDWESLNYLSNITPQKSHLNQGAWARLEDQERKLIDRADISSVYTVTGPLYERDMGKLPGTQKAHTIPSAYWKVIFINNSPAVNHYAAFLFDQNTPKGADFCQFRVTVDEIEKRTGLIIWAGLPDDVQASLKSKPGVLPELMGCKN

SEQ ID NO: 94 - protein, 245 aa, synthetic construct
  REGION 1..245: note = isolated from library
DTLESIDNCAVGCPTGGSSNVSIVRHAYTLNNNSTTKFANWVAYHITKDTLASGKLRNWKTDPALNPADTLAPADYTGANAALKVDRGHQAPLASLAGVSDWESLNYLSNITPQKSDLNQGAWARLEDQERKLIDRADISSVYTVTGPLYERDMGKLPGTQKAHTIPSAYWKVIFINNSPAVNHYAAFLFDQNTPKGADFCQFRVTVDEIEKRTGLIIWAGLPDDVQASLKSKPGVLPELMGCKN

SEQ ID NO: 95 - protein, 245 aa, synthetic construct
  REGION 1..245: note = isolated from library
DTLESIDNCAVGCPTGGSSNVSIVRHAYTLNNNSTTKFANWVAYHITKDTLASGKDRNWKTDPALNPADTLAPADYTGANAALKVDRGHQAPLASLAGVSDWESLNYLSNITPQKSDLNQGAWARLEDQERKLIDRADISSVYTVTGPLYERDMGKLPGTQKAHTIPSAYWKVIFINNSPAVNHYAAFLFDQNTPRGADFCQFRVTVDEIEKRTGLIIWAGLPDDVQASLKSKPGVLPELMGCKN

SEQ ID NO: 96 - protein, 245 aa, synthetic construct
  REGION 1..245: note = isolated from library
DTLESIDNCAVGCPTGGSSNVSIVRHAYTLNNNSTTKFANWVAYHITKDTLASGKMRNWKTDPALNPADTLAPADYTGANAALKVDRGHQAPLASLAGVSDWESLNYLSNITPQKSDLNQGAWARLEDQERKLIDRADISSVYTVTGPLYERDMGKLPGTQKAHTIPSAYWKVIFINNSPAVNHYAAFLFDQNTPKGADFCQFRVTVDEIEKRTGLIIWAGLPDDVQASLKSKPGVLPELMGCKN

SEQ ID NO: 97 - protein, 245 aa, synthetic construct
  REGION 1..245: note = isolated from library
DTLESIDNCAVGCPTGGSSNVSIVRHAYTLNNNSTTKFANWVAYHITKDTLASGKDRNWKTDPALNPADTLAPADYTGANAALKVDRGHQAPLASLAGVSDWESLNYLSNITPQKSYLNQGAWARLEDQERKLIDRADISSVYTVTGPLYERDMGKLPGTQKAHTIPSAYWKVIFINNSPAVNHYAAFLFDQNTPKGADFCQFRVTVDEIEKRTGLIIWAGLPDDVQASLKSKPGVLPELMGCKN

SEQ ID NO: 98 - protein, 245 aa, synthetic construct
  REGION 1..245: note = isolated from library
DTLESIDNCAVGCPTGGSSNVSIVRHAYTLNNNSTTKFANWVAYHITKDTLASGKDRNWKTDPALNPADTLAPADYTGANAALKVDRGHQAPLASLAGVSDWESLNYLSNITPQKSDLNQGAWARLEDQERKLIARADISSVYTVTGPLYERDMGKLPGTQKAHTIPSAYWKVIFINNSPAVNHYAAFLFDQNTPKGADFCQFRVTVDEIEKRTGLIIWAGLPDDVQASLKSKPGVLPELMGCKN

SEQ ID NO: 99 - protein, 245 aa, synthetic construct
  REGION 1..245: note = isolated from library
DTLESIDNCAVGCPTGGSSNVSIVRHAYTLNNNSTTKFANWVAYHITKDTLASGKDRNWKTDPALNPADTLAPADYTGANAALKVDRGHQAPLASLAGVSDWESLNYLSNITPQKSDLNQGAWARLEDQERKLIMRADISSVYTVTGPLYERDMGKLPGTQKAHTIPSAYWKVIFINNSPAVNHYAAFLFDQNTPKGADFCQFRVTVDEIEKRTGLIIWAGLPDDVQASLKSKPGVLPELMGCKN

SEQ ID NO: 100 - protein, 245 aa, synthetic construct
  REGION 1..245: note = isolated from library
DTLESIDNCAVGCPTGGSSNVSIVRHAYTLNNNSTTKFANWVAYHITKDTLASGKDRNWKTDPALNPADTLAPADYTGANAALKVDRGHQAPLASLAGVSDWESLNYLSNITPQKSDLNQGAWARLEDQERKLIDRADISSVYTVTGPLYERDMGKLPGTQKAHTIPSAYWKVIFINNSPAVNHYAAFLFDQNTPKGADFCQFQVTVDEIEKRTGLIIWAGLPDDVQASLKSKPGVLPELMGCKN

SEQ ID NO: 101 - protein, 245 aa, synthetic construct
  REGION 1..245: note = isolated from library
DTLESIDNCAVGCPTGGSSNVSIVRHAYTLNNNSTTKFANWVAYHITKDTLASGKDRNWKTDPALNPADTLAPADYTGAHAALKVDRGHQAPLASLAGVSDWESLNYLSNITPQKSDLNQGAWARLEDQERKLIDRADISSVYTVTGPLYERDMGKLPGTQKAHTIPSAYWKVIFINNSPAVNHYAAFLFDQNTPKGADFCQFRVTVDEIEKRTGLIIWAGLPDDVQASLKSKPGVLPELMGCKN

SEQ ID NO: 102 - protein, 245 aa, synthetic construct
  REGION 1..245: note = isolated from library
DTLESIDNCAVGCPTGGSSNVSIVRHAYTLNNNSTTKFANWVAYHITKDTLASGKDRNWKTDPALNPADTLAPADYTGANAALKVDRGHQAPLASLAGVSDWESLNYLSNITPQKSDLNQGAWARLEDQERKLIDRADISSVYTVTGPLYERDMGKLPGTQKAHTIPSAYWKVIFINNSPAVNHYAAFLFDQNTPKGADFCQFRVTVDEIEKRTGLIIWAGLPDDVQASLKSKPGVLPALMGCKN

SEQ ID NO: 103 - protein, 234 aa, Vibrio salmonicida
MKLIRLVISLIAVSFTVNVMAAPPSSFSKAKKEAVKIYLDYPTSFYCGCDITWKNKKKGIPELESCGYQVRKQEKRASRIEWEHVVPAWQFGHQRQCWQKGGRKNCTRNDKQFKSMEADLHNLVPAIGEVNGDRSNFRFSQWNGSKGAFYGQCAFKVDFKGRVAEPPAQSRGAIARTYLYMNNEYKFNLSKAQRQLMEAWNKQYPVSTWECTRDERIAKIQGNHNQFVYKACTK

SEQ ID NO: 104 - protein, 265 aa, Serratia ficaria
MRLNKMLALATLLLAAQASAETLESIDNCAVGCPTGGSSNMSLVRHAYTLNNNSTTKFANWVAYHITKETPASGKTRNWKTDPALNPADTLAPADYTGANAALKVDRGHQAPLASLAGVSDWESLNYLSNITPQKSDLNQGSWARLEDQERRLIERADVSSVYTVTGPLFERDMGKLPGTQKAHTIPSAYWKVIFINNSPAVNHYAAFLFDQDTPKNADFCQYRVTVDEIEKRSGLIIWAGLPEDVQASLKSKPGVLPELMGCKN

SEQ ID NO: 105 - protein, 265 aa, Serratia odorifera
MRLSRIIALSALLLATQAGAATLESIDNCAVGCPTGGDSNLSIVRHAYTLNNNGDTKFANWVAYHITKDTLASGKSRTWRTDPALDPAQTLAPADYTGANAALQVDRGHQAPLASLANVSDWESLNYLSNITPQKSDLNQGSWAALEDQERKLIARADISSVYTVTGPLYERDMGKLPGTTKSHTIPSGYWKVIFINNSPEVNHYAAFIFDQNTPRGADFCQFRVTVDEVEKRSGLILWAGLPDDVQATLKQKPGVLPELMGCQR

SEQ ID NO: 106 - protein, 245 aa, synthetic construct
  REGION 1..245: note = isolated from library
DTLESIDNCAVGCPTGGSSNVSIVRHAYTLNNNSTTKFANWVAYHITKDTPASGKTRNWKTDPALNPADTLAPADYTGANAALKVDRGHQAPLASLAGVSDWESLNYLSNITPQKSDLNQGAWARLEDQERKLIDRADISSVYTVTGPLYERDMGKLPGTQKAHTIPSAYWKVIFINNSPAVNHYAAFLFDQNTPKGADFCQFRVTVDEIEKRTGLIFWAGLPDDVQASLKSKPGVLPELMGCKN

SEQ ID NO: 107 - protein, 245 aa, synthetic construct
  REGION 1..245: note = isolated from library
DTLESIDNCAVGCPTGGSSNVSIVRHAYTLNNNSTTKFANWVAYHITKDTPASGKTRNWKTDPALNPADTLAPADYTGANAALKVDRGHQAPLASLAGVSDWESLNYLSNITPQKSDLNQGAWARLEDQERRLIDRADISSVYTVTGPLYERDMGKLPGTQKAHTIPSAYWKVIFINNSPAVNHYAAFLFDQNTPKGADFCQFRVTVDEIEKRTGLIIWAGLPDDVQASLKSKPGVLPELMGCKN

SEQ ID NO: 108 - protein, 245 aa, synthetic construct
  REGION 1..245: note = isolated from library
DTLESIDNCAVGCPTGGSSNVSIVRHAYTLNNNSTTKFANWVAYHITKDTPASGKTRNWKTDPALNPADTLAPADYTGANAALKVDRGHQAPLASLAGVSDWESLNYLSNITPQKSDLNQGAWARLEDQERKLIDRADISSVYTVTGPLYLRDMGKLPGTQKAHTIPSAYWKVIFINNSPAVNHYAAFLFDQNTPKGADFCQFRVTVDEIEKRTGLIIWAGLPDDVQASLKSKPGVLPELMGCKN

SEQ ID NO: 109 - protein, 245 aa, synthetic construct
  REGION 1..245: note = isolated from library
DTLESIDNCAVGCPTGGSSNVSIVRHAYTLNNNSTTKFANWVAYHITKDTPASGKTRNWKTDPALNPADTLAPADYTGANAALKVDRGHQAPLGSLAGVSDWESLNYLSNITPQKSDLNQGAWARLEDQERKLIDRADISSVYTVTGPLYERDMGKLPGTQKAHTIPSAYWKVIFINNSPAVNHYAAFLFDQNTPKGADFCQFRVTVDEIEKRTGLIIWAGLPDDVQASLKSKPGVLPELMGCKN

SEQ ID NO: 110 - protein, 245 aa, synthetic construct
  REGION 1..245: note = isolated from library
DTLESIDNCAVGCPTGGSSNVSIVRHAYTLNNNSTTKFANWVAYHITKDTPASGKTRNWKTDPALNPADTLAPADYTGANAALKVDRGHQAPLASLAGVSDWESLNYLSNITPQKSDLNQGAWARLEDQERKLIDRADISSVYTVTGPLYERDMGKLPGTQNAHTIPSAYWKVIFINNSPAVNHYAAFLFDQNTPKGADFCQFRVTVDEIEKRTGLIIWAGLPDDVQASLKSKPGVLPELMGCKN

SEQ ID NO: 111 - protein, 245 aa, synthetic construct
  REGION 1..245: note = isolated from library
DTLESIDNCAVGCPTGGSSNVSIVRHAYTLNNNSTTKFANWVAYHITKDTPASGKTRNWKTDPALNPADTLAPADYTGANAALKVDRGHQAPLASLAGVSDWESLNYLSNITPQKSDLNQGAWARLEDQERKLIDRADISSVYTVTGPLYERDMGKLPGTQKAHTIPSAYWKVIFINNSPAVNHYAAFLFDQNTPKGADFCQFRVTVDEIEKRTGLIIWAGLPDDVQRSLKSKPGVLPELMGCKN

SEQ ID NO: 112 - protein, 245 aa, synthetic construct
  REGION 1..245: note = isolated from library
DTLESIDNCAVGCPTGGSSNVSIVRHAYTLNNNSTTKFANWVAYHITKDTPASGKTRNWKTDPALNPADTLAPADYTRANAALKVDRGHQAPLASLAGVSDWESLNYLSNITPQKSDLNQGAWARLEDQERKLIDRADISSVYTVTGPLYERDMGKLPGTQKAHTIPSAYWKVIFINNSPAVNHYAAFLFDQNTPKGADFCQFRVTVDEIEKRTGLIIWAGLPDDVQASLKSKPGVLPELMGCKN

SEQ ID NO: 113 - protein, 245 aa, synthetic construct
  REGION 1..245: note = isolated from library
DTLESIDNCAVGCPTGGSSNVSIVRHAYTLNNNSTTKFANWVAYHITKDTPASGKTRNWKTDPALNPADTLAPADYTGANKALKVDRGHQAPLASLAGVSDWESLNYLSNITPQKSDLNQGAWARLEDQERKLIDRADISSVYTVTGPLYERDMGKLPGTQKAHTIPSAYWKVIFINNSPAVNHYAAFLFDQNTPKGADFCQFRVTVDEIEKRTGLIIWAGLPDDVQASLKSKPGVLPELMGCKN

SEQ ID NO: 114 - protein, 245 aa, synthetic construct
  REGION 1..245: note = isolated from library
DTLESIDNCAVGCPTGGSSNVSIVRHAYTLNNNSTTKFANWVAYHITKDTPASGKTRNWKTDPALNPADTLAPADYTGANAALKVDRGHQAPLASLAGVSDWESLNYLSNITPQKSDLNRGAWARLEDQERKLIDRADISSVYTVTGPLYERDMGKLPGTQKAHTIPSAYWKVIFINNSPAVNHYAAFLFDQNTPKGADFCQFRVTVDEIEKRTGLIIWAGLPDDVQASLKSKPGVLPELMGCKN

SEQ ID NO: 115 - protein, 245 aa, synthetic construct
  REGION 1..245: note = isolated from library
DTLESIDNCAVGCPTGGSSNVSIVRHAYTLNNNSTTKFANWVAYHITKDTPASGKTRNWKTDPALNPADTLAPADYTGANARLKVDRGHQAPLASLAGVSDWESLNYLSNITPQKSDLNQGAWARLEDQERKLIDRADISSVYTVTGPLYERDMGKLPGTQKAHTIPSAYWKVIFINNSPAVNHYAAFLFDQNTPKGADFCQFRVTVDEIEKRTGLIIWAGLPDDVQASLKSKPGVLPELMGCKN

SEQ ID NO: 116 - protein, 245 aa, synthetic construct
  REGION 1..245: note = isolated from library
DTLESIDNCAVGCPTGGSSNVSIVRHAYTLNNNSTTKFANWVAYHITKDTPASGKTRNWKTDPALNPADTLAPADYTGANAALKVDRGHQAPLASLAGVSDWESLNYLSNITPQKSDLNQGAWARLEDQERKLIARADISSVYTVTGPLYERDMGKLPGTQKAHTIPSAYWKVIFINNSPAVNHYAAFLFDQNTPKGADFCQFRVTVDEIEKRTGLIIWAGLPDDVQASLKSKPGVLPELMGCKN

SEQ ID NO: 117 - protein, 245 aa, synthetic construct
  REGION 1..245: note = isolated from library
DTLESIDNCAVGCPTGGSSNVSIVRHAYTLNNNSTTKFANWVAYHITKDTPASGKTRNWKTDPALNPADTLAPADYTGANAALKVDRGHQAPLASLAGVSDWESLNYLSNITPQKSDLNQGAWARLEDQERKLIDRADISSVYTVTGPLYERDMGKLPGTQKAHTIPSAYWKVIFINNSPAVNHYAAFLFDQNTPRGADFCQFRVTVDEIEKRTGLIIWAGLPDDVQASLKSKPGVLPELMGCKN

SEQ ID NO: 118 - protein, 245 aa, synthetic construct
  REGION 1..245: note = isolated from library
DTLESIDNCAVGCPTGGSSNVSIVRHAYTLNNNSTTKFANWVAYHITKDTPASGKSRNWKTDPALNPADTLAPADYTGANAALKVDRGHQAPLASLAGVSDWESLNYLSNITPQKSDLNQGAWARLEDQERKLIDRADISSVYTVTGPLYERDMGKLPGTQKAHTIPSAYWKVIFINNSPAVNHYAAFLFDQNTPKGADFCQFRVTVDEIEKRTGLIIWAGLPDDVQASLKSKPGVLPELMGCKN

SEQ ID NO: 119 - protein, 245 aa, synthetic construct
  REGION 1..245: note = isolated from library
DTLESIDNCAVGCPTGGSSNVSIVRHAYTLNNNSTTKFANWVAYHITKDTPASGKGRNWKTDPALNPADTLAPADYTGANAALKVDRGHQAPLASLAGVSDWESLNYLSNITPQKSDLNQGAWARLEDQERKLIDRADISSVYTVTGPLYERDMGKLPGTQKAHTIPSAYWKVIFINNSPAVNHYAAFLFDQNTPKGADFCQFRVTVDEIEKRTGLIIWAGLPDDVQASLKSKPGVLPELMGCKN

SEQ ID NO: 120 - protein, 245 aa, synthetic construct
  REGION 1..245: note = isolated from library
DTLESIDNCAVGCPTGGSSNVSIVRHAYTLNNNSTTKFANWVAYHITKDTLASGKGRNWKTDPALNPADTLAPADYTGANKALKVDRGHQAPLASLAGVSDWESLNYLSNITPQKSDLNQGAWARLEDQERKLIDRADISSVYTVTGPLYERDMGKLPGTQKAHTIPSAYWKVIFINNSPAVNHYAAFLFDQNTPKGADFCQFRVTVDEIEKRTGLIIWAGLPDDVQASLKSKPGVLPELMGCKN

SEQ ID NO: 121 - protein, 245 aa, synthetic construct
  REGION 1..245: note = isolated from library
DTLESIDNCAVGCPTGGSSNVSIVRHAYTLNNNSTTKFANWVAYHITKDTLASGKKRNWKTDPALNPADTLAPADYTGANAALKVDRGHQAPLASLAGVSDWESLNYLSNITPQKSDLNQGAWARLEDQERKLIARADISSVYTVTGPLYERDMGKLPGTQKAHTIPSAYWKVIFINNSPAVNHYAAFLFDQNTPKGADFCQFRVTVDEIEKRTGLIIWAGLPDDVQASLKSKPGVLPELMGCKN

SEQ ID NO: 122 - protein, 245 aa, synthetic construct
  REGION 1..245: note = isolated from library
DTLESIDNCAVGCPTGGSSNVSIVRHAYTLNNNSTTKFANWVAYHITKDTLASGKPRNWKTDPALNPADTLAPADYTGANAALKVDRGHQAPLASLAGVSDWESLNYLSNITPQKSDLNQGAWKRLEDQERKLIDRADISSVYTVTGPLYERDMGKLPGTQKAHTIPSAYWKVIFINNSPAVNHYAAFLFDQNTPKGADFCQFRVTVDEIEKRTGLIIWAGLPDDVQASLKSKPGVLPELMGCKN

SEQ ID NO: 123 - protein, 245 aa, synthetic construct
  REGION 1..245: note = isolated from library
DTLESIDNCAVGCPTGGSSNVSIVRHAYTLNNNSTTKFANWVAYHITKDTLASGKPRNWKTDPALNPADTLAPADYTGANAALKVDRGHQAPLASLAGVSDWESLNYLSNITPQKSDLNQGAWARLEDQERKLIARADISSVYTVTGPLYERDMGKLPGTQKAHTIPSAYWKVIFINNSPAVNHYAAFLFDQNTPKGADFCQFRVTVDEIEKRTGLIIWAGLPDDVQASLKSKPGVLPELMGCKN

SEQ ID NO: 124 - protein, 245 aa, synthetic construct
  REGION 1..245: note = isolated from library
DTLESIDNCAVGCPTGGSSNVSIVRHAYTLNNNSTTKFANWVAYHITKDTLASGKSRNWKTDPALNPADTLAPADYTGANKALKVDRGHQAPLASLAGVSDWESLNYLSNITPQKSDLNQGAWARLEDQERKLIDRADISSVYTVTGPLYERDMGKLPGTQKAHTIPSAYWKVIFINNSPAVNHYAAFLFDQNTPKGADFCQFRVTVDEIEKRTGLIIWAGLPDDVQASLKSKPGVLPALMGCKN

SEQ ID NO: 125 - protein, 245 aa, synthetic construct
  REGION 1..245: note = isolated from library
DTLESIDNCAVGCPTGGSSNVSIVRHAYTLNNNSTTKFANWVAYHITKDTLASGKDRNWKTDPALNPADTLAPADYTGANAALKVDRGHQAPLASLAGVSDWESLNYLSNITPQKSDLNRGAWKRLEDQERKLIDRADISSVYTVTGPLYERDMGKLPGTQKAHTIPSAYWKVIFINNSPAVNHYAAFLFDQNTPKGADFCQFRVTVDEIEKRTGLIIWAGLPDDVQASLKSKPGVLPELMGCKN

SEQ ID NO: 126 - protein, 245 aa, synthetic construct
  REGION 1..245: note = isolated from library
DTLESIDNCAVGCPTGGSSNVSIVRHAYTLNNNSTTKFANWVAYHITKDTLASGKDRNWKTDPALNPADTLAPADYTGANKALKVDRGHQAPLASLAGVSDWESLNYLSNITPQKSDLNQGAWKRLEDQERKLIDRADISSVYTVTGPLYERDMGKLPGTQKAHTIPSAYWKVIFINNSPAVNHYAAFLFDQNTPKGADFCQFRVTVDEIEKRTGLIIWAGLPDDVQASLKSKPGVLPELMGCKN

SEQ ID NO: 127 - protein, 245 aa, synthetic construct
  REGION 1..245: note = isolated from library
DTLESIDNCAVGCPTGGSSNVSIVRHAYTLNNNSTTKFANWVAYHITKDTLASGKKRNWKTDPALNPADTLAPADYTGANKALKVDRGHQAPLASLAGVSDWESLNYLSNITPQKSDLNQGAWKRLEDQERKLIDRADISSVYTVTGPLYERDMGKLPGTQKAHTIPSAYWKVIFINNSPAVNHYAAFLFDQNTPKGADFCQFRVTVDEIEKRTGLIIWAGLPDDVQASLKSKPGVLPELMGCKN

SEQ ID NO: 128 - protein, 245 aa, synthetic construct
  REGION 1..245: note = isolated from library
DTLESIDNCAVGCPTGGSSNVSIVRHAYTLNNNSTTKFANWVAYHITKDTLASGKGRNWKTDPALNPADTLAPADYKGANKALKVDRGHQAPLASLAGVSDWESLNYLSNITPQKSDLNQGAWARLEDQERKLIDRADISSVYTVTGPLYERDMGKLPGTQKAHTIPSAYWKVIFINNSPAVNHYAAFLFDQNTPKGADFCQFRVTVDEIEKRTGLIIWAGLPDDVQASLKSKPGVLPALMGCKN

SEQ ID NO: 129 - protein, 245 aa, synthetic construct
  REGION 1..245: note = isolated from library
DTLESIDNCAVGCPTGGSSNVSIVRHAYTLNNNSTTKFANWVAYHITKDTLASGKDRNWKTDPALNPADTLAPADYTGANKALKVDRGHQAPLASLAGVSDWESLNYLSNITPQKSDLNQGAWKRLEDQERKLIDRADISSVYTVTGPLYERDMGKLPGTQKAHTIPSAYWKVIFINNSPAVNHYAAFLFDQNTPKGADFCQFRVTVDEIEKRTGLIIWAGLPDDVQASLKSKPGVLPALMGCKN

SEQ ID NO: 130 - protein, 245 aa, synthetic construct
  REGION 1..245: note = isolated from library
DTLESIDNCAVGCPTGGSSNVSIVRHAYTLNNNSTTKFANWVAYHITKDTLASGKDRNWKTDPALNPADTLAPADYTGANKALKVDRGHQAPLASLAGVSDWESLNYLSNITPQKSDLNQGAWARLEDQERKLIARADISSVYTVTGPLYERDMGKLPGTQKAHTIPSAYWKVIFINNSPAVNHYAAFLFDQNTPKGADFCQFRVTVDEIEKRTGLIIWAGLPDDVQASLKSKPGVLPALMGCKN

SEQ ID NO: 131 - protein, 245 aa, synthetic construct
  REGION 1..245: note = isolated from library
DTLESIDNCAVGCPTGGSSNVSIVRHAYTLNNNSTTKFANWVAYHITKDTLASGKGRNWKTDPALNPADTLAPADYKGANAALKVDRGHQAPLASLAGVSDWESLNYLSNITPQKSDLNQGAWARLEDQERKLIARADISSVYTVTGPLYERDMGKLPGTQKAHTIPSAYWKVIFINNSPAVNHYAAFLFDQNTPKGADFCQFRVTVDEIEKRTGLIIWAGLPDDVQASLKSKPGVLPALMGCKN

SEQ ID NO: 132 - protein, 245 aa, synthetic construct
  REGION 1..245: note = isolated from library
DTLESIDNCAVGCPTGGSSNVSIVRHAYTLNNNSTTKFANWVAYHITKDTLASGKDRNWKTDPALNPADTLAPADYKGANAALKVDRGHQAPLASLAGVSDWESLNYLSNITPQKSDLNRGAWARLEDQERKLIARADISSVYTVTGPLYERDMGKLPGTQKAHTIPSAYWKVIFINNSPAVNHYAAFLFDQNTPKGADFCQFRVTVDEIEKRTGLIIWAGLPDDVQASLKSKPGVLPELMGCKN

SEQ ID NO: 133 - protein, 245 aa, synthetic construct
  REGION 1..245: note = isolated from library
DTLESIDNCAVGCPTGGSSNVSIVRHAYTLNNNSTTKFANWVAYHITKDTLASGKKRNWKTDPALNPADTLAPADYKGANKALKVDRGHQAPLASLAGVSDWESLNYLSNITPQKSDLNQGAWARLEDQERKLIARADISSVYTVTGPLYERDMGKLPGTQKAHTIPSAYWKVIFINNSPAVNHYAAFLFDQNTPKGADFCQFRVTVDEIEKRTGLIIWAGLPDDVQASLKSKPGVLPELMGCKN

SEQ ID NO: 134 - protein, 245 aa, synthetic construct
  REGION 1..245: note = isolated from library
DTLESIDNCAVGCPTGGSSNVSIVRHAYTLNNNSTTKFANWVAYHITKDTLASGKSRNWKTDPALNPADTLAPADYKGANKALKVDRGHQAPLASLAGVSDWESLNYLSNITPQKSDLNQGAWARLEDQERKLIARADISSVYTVTGPLYERDMGKLPGTQKAHTIPSAYWKVIFINNSPAVNHYAAFLFDQNTPKGADFCQFRVTVDEIEKRTGLIIWAGLPDDVQASLKSKPGVLPELMGCKN

SEQ ID NO: 135 - protein, 245 aa, synthetic construct
  REGION 1..245: note = isolated from library
DTLESIDNCAVGCPTGGSSNVSIVRHAYTLNNNSTTKFANWVAYHITKDTLASGKGRNWKTDPALNPADTLAPADYTGANAALKVDRGHQAPLASLAGVSDWESLNYLSNITPQKSDLNRGAWKRLEDQERKLIARADISSVYTVTGPLYERDMGKLPGTQKAHTIPSAYWKVIFINNSPAVNHYAAFLFDQNTPKGADFCQFRVTVDEIEKRTGLIIWAGLPDDVQASLKSKPGVLPELMGCKN

SEQ ID NO: 136 - protein, 245 aa, synthetic construct
  REGION 1..245: note = isolated from library
DTLESIDNCAVGCPTGGSSNVSIVRHAYTLNNNSTTKFANWVAYHITKDTLASGKDRNWKTDPALNPADTLAPADYTGANKALKVDRGHQAPLASLAGVSDWESLNYLSNITPQKSHLNQGAWKRLEDQERKLIDRADISSVYTVTGPLYERDMGKLPGTQKAHTIPSAYWKVIFINNSPAVNHYAAFLFDQNTPKGADFCQFRVTVDEIEKRTGLIIWAGLPDDVQASLKSKPGVLPELMGCKN

SEQ ID NO: 137 - protein, 245 aa, synthetic construct
  REGION 1..245: note = isolated from library
DTLESIDNCAVGCPTGGSSNVSIVRHAYTLNNNSTTKFANWVAYHITKDTLASGKSRNWKTDPALNPADTLAPADYKGANKALKVDRGHQAPLASLAGVSDWESLNYLSNITPQKSDLNQGAWARLEDQERKLIARADISSVYTVTGPLYERDMGKLPGTQKAHTIPSAYWKVIFINNSPAVNHYAAFLFDQNTPKGADFCQFRVTVDEIEKRTGLIIWAGLPDDVQASLKSKPGVLPALMGCKN

SEQ ID NO: 138 - protein, 245 aa, synthetic construct
  REGION 1..245: note = isolated from library
DTLESIDNCAVGCPTGGSSNVSIVRHAYTLNNNSTTKFANWVAYHITKDTLASGKDRNWKTDPALNPADTLAPADYKGANKALKVDRGHQAPLASLAGVSDWESLNYLSNITPQKSHLNQGAWARLEDQERKLIARADISSVYTVTGPLYERDMGKLPGTQKAHTIPSAYWKVIFINNSPAVNHYAAFLFDQNTPKGADFCQFRVTVDEIEKRTGLIIWAGLPDDVQASLKSKPGVLPELMGCKN

SEQ ID NO: 139 - protein, 245 aa, synthetic construct
  REGION 1..245: note = isolated from library
DTLESIDNCAVGCPTGGSSNVSIVRHAYTLNNNSTTKFANWVAYHITKDTLASGKDRNWKTDPALNPADTLAPADYKGANAALKVDRGHQAPLASLAGVSDWESLNYLSNITPQKSDLNRGAWARLENQERKLIARADISSVYTVTGPLYERDMGKLPGTQKAHTIPSAYWKVIFINNSPAVNHYAAFLFDQNTPKGADFCQFRVTVDEIEKRTGLIIWAGLPDDVQASLKSKPGVLPELMGCKN

SEQ ID NO: 140 - protein, 245 aa, synthetic construct
  REGION 1..245: note = isolated from library
DTLESIDNCAVGCPTGGSSNVSIVRHAYTLNNNSTTKFANWVAYHITKDTLASGKDRNWKTDPALNPADTLAPADYKGANKALKVDRGHQAPLASLAGVSDWESLNYLSNITPQKSDLNRGAWARLEDQERKLIARADISSVYTVTGPLYERDMGKLPGTQKAHTIPSAYWKVIFINNSPAVNHYAAFLFDQNTPKGADFCQFRVTVDEIEKRTGLIIWAGLPDDVQASLKSKPGVLPELMGCKN

SEQ ID NO: 141 - protein, 245 aa, synthetic construct
  REGION 1..245: note = isolated from library
DTLESIDNCAVGCPTGGSSNVSIVRHAYTLNNNSTTKFANWVAYHITKDTLASGKDRNWKTDPALNPADTLAPADYTGANKALKVDRGHQAPLASLAGVSDWESLNYLSNITPQKSDLNRGAWKRLEDQERKLIARADISSVYTVTGPLYERDMGKLPGTQKAHTIPSAYWKVIFINNSPAVNHYAAFLFDQNTPKGADFCQFRVTVDEIEKRTGLIIWAGLPDDVQASLKSKPGVLPELMGCKN

SEQ ID NO: 142 - protein, 245 aa, synthetic construct
  REGION 1..245: note = isolated from library
DTLESIDNCAVGCPTGGSSNVSIVRHAYTLNNNSTTKFANWVAYHITKDTLASGKDRNWKTDPALNPADTLAPADYTGANKALKVDRGHQAPLASLAGVSDWESLNYLSNITPQKSDLNRGAWKRLEDQERKLIARADISSVYTVTGPLYERDMGKLPGTQKAHTIPSAYWKVIFINNSPAVNHYAAFLFDQNTPKGADFCQFRVTVDEIEKRTGLIIWAGLPDDVQASLKSKPGVLPALMGCKN

SEQ ID NO: 143 - protein, 245 aa, synthetic construct
  REGION 1..245: note = isolated from library
DTLESIDNCAVGCPTGGSSNVSIVRHAYTLNNNSTTKFANWVAYHITKDTLASGKDRNWKTDPALNPADTLAPADYKGANKALKVDRGHQAPLASLAGVSDWESLNYLSNITPQKSDLNRGAWKRLEDQERKLIARADISSVYTVTGPLYERDMGKLPGTQKAHTIPSAYWKVIFINNSPAVNHYAAFLFDQNTPKGADFCQFRVTVDEIEKRTGLIIWAGLPDDVQASLKSKPGVLPELMGCKN

SEQ ID NO: 144 - protein, 245 aa, synthetic construct
  REGION 1..245: note = isolated from library
DTLESIDNCAVGCPTGGSSNVSIVRHAYTLNNNSTTKFANWVAYHITKDTLASGKDRNWKTDPALNPADTLAPADYTGANKALKVDRGHQAPLASLAGVSDWESLNYLSNITPQKSDLNQGAWARLEDQERKLIDRADISSVYTVTGPLYERDMGKLPGTQKAHTIPSAYWKVIFINNSPAVNHYAAFLFDQNTPKGADFCQFRVTVDEIEKRTGLIIWAGLPDDVQASLKSKPGVLPELMGCKN

SEQ ID NO: 145 - protein, 245 aa, synthetic construct
  REGION 1..245: note = isolated from library
DTLESIDNCAVGCPTGGSSNVSIVRHAYTLNNNSTTKFANWVAYHITKDTPRSGKTRNWKTDPALNPADTLAPADYTGANAALKVDRGHQAPLASLAGVSDWESLNYLSNITPQKSDLNQGAWARLEDQERKLIDRADISSVYTVTGPLYERDMGKLPGTQKAHTIPSAYWKVIFINNSPAVNHYAAFLFDQNTPKGADFCQFRVTVDEIEKRTGLIIWAGLPDDVQASLKSKPGVLPELMGCKN

SEQ ID NO: 146 - protein, 245 aa, synthetic construct
  REGION 1..245: note = isolated from library
DTLESIDNCAVGCPTGGSSNVSIVRHAYTLNNNSTTKFANWVAYHITKDTPASRKTRNWKTDPALNPADTLAPADYTGANAALKVDRGHQAPLASLAGVSDWESLNYLSNITPQKSDLNQGAWARLEDQERKLIDRADISSVYTVTGPLYERDMGKLPGTQKAHTIPSAYWKVIFINNSPAVNHYAAFLFDQNTPKGADFCQFRVTVDEIEKRTGLIIWAGLPDDVQASLKSKPGVLPELMGCKN

SEQ ID NO: 147 - protein, 245 aa, synthetic construct; identical to SEQ ID NO: 18
  REGION 1..245: note = isolated from library

SEQ ID NO: 148 - protein, 245 aa, synthetic construct; identical to SEQ ID NO: 19
  REGION 1..245: note = isolated from library

SEQ ID NO: 149 - protein, 245 aa, synthetic construct; identical to SEQ ID NO: 112
  REGION 1..245: note = isolated from library

SEQ ID NO: 150 - protein, 245 aa, synthetic construct
  REGION 1..245: note = isolated from library
DTLESIDNCAVGCPTGGSSNVSIVRHAYTLNNNSTTKFANWVAYHITKDTPASGKTRNWKTDPALNPADTLAPADYTGARAALKVDRGHQAPLASLAGVSDWESLNYLSNITPQKSDLNQGAWARLEDQERKLIDRADISSVYTVTGPLYERDMGKLPGTQKAHTIPSAYWKVIFINNSPAVNHYAAFLFDQNTPKGADFCQFRVTVDEIEKRTGLIIWAGLPDDVQASLKSKPGVLPELMGCKN

SEQ ID NO: 151 - protein, 245 aa, synthetic construct
  REGION 1..245: note = isolated from library
DTLESIDNCAVGCPTGGSSNVSIVRHAYTLNNNSTTKFANWVAYHITKDTPASGKTRNWKTDPALNPADTLAPADYTGANAALKVDRGHQAPLASLAGVSDWESLNYLSNITPQKSDLRQGAWARLEDQERKLIDRADISSVYTVTGPLYERDMGKLPGTQKAHTIPSAYWKVIFINNSPAVNHYAAFLFDQNTPKGADFCQFRVTVDEIEKRTGLIIWAGLPDDVQASLKSKPGVLPELMGCKN

SEQ ID NO: 152 - protein, 245 aa, synthetic construct
  REGION 1..245: note = isolated from library
DTLESIDNCAVGCPTGGSSNVSIVRHAYTLNNNSTTKFANWVAYHITKDTPASGKTRNWKTDPALNPADTLAPADYTGANAALKVDRGHQAPLASLAGVSDWESLNYLSNITPQKSDLNQGAWARLEDQERKLIDRADISSVYTVTGPLYERDMGKLPGTQKAHTIPSAYWKVIFINNSPAVNHYAAFLFDQNTRKGADFCQFRVTVDEIEKRTGLIIWAGLPDDVQASLKSKPGVLPELMGCKN

SEQ ID NO: 153 - protein, 245 aa, synthetic construct
  REGION 1..245: note = isolated from library
DTLESIDNCAVGCPTGGSSNVSIVRHAYTLNNNSTTKFANWVAYHITKDTLASGKTRNWKTDPALNPADTLAPADYRGANAALKVDRGHQAPLASLAGVSDWESLNYLSNITPQKSDLNQGAWARLEDQERKLIDRADISSVYTVTGPLYERDMGKLPGTQKAHTIPSAYWKVIFINNSPAVNHYAAFLFDQNTPKGADFCQFRVTVDEIEKRTGLIIWAGLPDDVQASLKSKPGVLPELMGCKN

SEQ ID NO: 154 - protein, 245 aa, synthetic construct
  REGION 1..245: note = isolated from library
DTLESIDNCAVGCPTGGSSNVSIVRHAYTLNNNSTTKFANWVAYHITKDTLASGKTRNWKTDPALNPADTLAPADYKGANAALKVDRGHQAPLASLAGVSDWESLNYLSNITPQKSDLNQGAWARLEDQERKLIDRADISSVYTVTGPLYERDMGKLPGTQKAHTIPSAYWKVIFINNSPAVNHYAAFLFDQNTPKGADFCQFRVTVDEIEKRTGLIIWAGLPDDVQASLKSKPGVLPELMGCKN

SEQ ID NO: 155 - protein, 245 aa, synthetic construct
  REGION 1..245: note = isolated from library
DTLESIDNCAVGCPTGGSSNVSIVRHAYTLNNNSTTKFANWVAYHITKDTGASGKTRNWKTDPALNPADTLAPADYKGANAALKVDRGHQAPLASLAGVSDWESLNYLSNITPQKSDLNQGAWARLEDQERKLIDRADISSVYTVTGPLYERDMGKLPGTQKAHTIPSAYWKVIFINNSPAVNHYAAFLFDQNTPKGADFCQFRVTVDEIEKRTGLIIWAGLPDDVQASLKSKPGVLPELMGCKN

SEQ ID NO: 156 - protein, 245 aa, synthetic construct
  REGION 1..245: note = isolated from library
DTLESIDNCAVGCPTGGSSNVSIVRHAYTLNNNSTTKFANWVAYHITKDTGASGKTRNWKTDPALNPADTLAPADYRGANAALKVDRGHQAPLASLAGVSDWESLNYLSNITPQKSDLNQGAWARLEDQERKLIDRADISSVYTVTGPLYERDMGKLPGTQKAHTIPSAYWKVIFINNSPAVNHYAAFLFDQNTPKGADFCQFRVTVDEIEKRTGLIIWAGLPDDVQASLKSKPGVLPELMGCKN

SEQ ID NO: 157 - protein, 245 aa, synthetic construct
  REGION 1..245: note = isolated from library
DTLESIDNCAVGCPTGGSSNVSIVRHAYTLNNNSTTKFANWVAYHITKDTLASGKTRNWKTDPALNPADTLAPADYHGANAALKVDRGHQAPLASLAGVSDWESLNYLSNITPQKSDLNQGAWARLEDQERKLIDRADISSVYTVTGPLYERDMGKLPGTQKAHTIPSAYWKVIFINNSPAVNHYAAFLFDQNTPKGADFCQFRVTVDEIEKRTGLIIWAGLPDDVQASLKSKPGVLPELMGCKN

SEQ ID NO: 158 - protein, 245 aa, synthetic construct
  REGION 1..245: note = isolated from library
DTLESIDNCAVGCPTGGSSNVSIVRHAYTLNNNSTTKFANWVAYHITKDTGASGKTRNWKTDPALNPADTLAPADYHGANAALKVDRGHQAPLASLAGVSDWESLNYLSNITPQKSDLNQGAWARLEDQERKLIDRADISSVYTVTGPLYERDMGKLPGTQKAHTIPSAYWKVIFINNSPAVNHYAAFLFDQNTPKGADFCQFRVTVDEIEKRTGLIIWAGLPDDVQASLKSKPGVLPELMGCKN

SEQ ID NO: 159 - protein, 245 aa, synthetic construct
  REGION 1..245: note = isolated from library
DTLESIDNCAVGCPTGGSSNVSIVRHAYTLNNNSTTKFANWVAYHITKDTAASGKTRNWKTDPALNPADTLAPADYRGANAALKVDRGHQAPLASLAGVSDWESLNYLSNITPQKSDLNQGAWARLEDQERKLIDRADISSVYTVTGPLYERDMGKLPGTQKAHTIPSAYWKVIFINNSPAVNHYAAFLFDQNTPKGADFCQFRVTVDEIEKRTGLIIWAGLPDDVQASLKSKPGVLPELMGCKN

SEQ ID NO: 160 - protein, 245 aa, synthetic construct
  REGION 1..245: note = isolated from library
DTLESIDNCAVGCPTGGSSNVSIVRHAYTLNNNSTTKFANWVAYHITKDTVASGKTRNWKTDPALNPADTLAPADYRGANAALKVDRGHQAPLASLAGVSDWESLNYLSNITPQKSDLNQGAWARLEDQERKLIDRADISSVYTVTGPLYERDMGKLPGTQKAHTIPSAYWKVIFINNSPAVNHYAAFLFDQNTPKGADFCQFRVTVDEIEKRTGLIIWAGLPDDVQASLKSKPGVLPELMGCKN

SEQ ID NO: 161 - protein, 245 aa, synthetic construct
  REGION 1..245: note = isolated from library
DTLESIDNCAVGCPTGGSSNVSIVRHAYTLNNNSTTKFANWVAYHITKDTIASGKTRNWKTDPALNPADTLAPADYRGANAALKVDRGHQAPLASLAGVSDWESLNYLSNITPQKSDLNQGAWARLEDQERKLIDRADISSVYTVTGPLYERDMGKLPGTQKAHTIPSAYWKVIFINNSPAVNHYAAFLFDQNTPKGADFCQFRVTVDEIEKRTGLIIWAGLPDDVQASLKSKPGVLPELMGCKN

SEQ ID NO: 162 - protein, 245 aa, synthetic construct
  REGION 1..245: note = isolated from library
DTLESIDNCAVGCPTGGSSNVSIVRHAYTLNNNSTTKFANWVAYHITKDTLASGKTRNWKTDPALNPADTLAPADYRGANAALKVDRGHQAPLASLAGVSDWESLNYLSNITPQKSDLNQGAWHRLEDQERKLIDRADISSVYTVTGPLYERDMGKLPGTQKAHTIPSAYWKVIFINNSPAVNHYAAFLFDQNTPKGADFCQFRVTVDEIEKRTGLIIWAGLPDDVQASLKSKPGVLPELMGCKN

SEQ ID NO: 163 - protein, 245 aa, synthetic construct
  REGION 1..245: note = isolated from library
DTLESIDNCAVGCPTGGSSNVSIVRHAYTLNNNSTTKFANWVAYHITKDTLASGKTRNWKTDPALNPADTLAPADYRGANAALKVDRGHQAPLASLAGVSDWESLNYLSNITPQKSDLNQGAWRRLEDQERKLIDRADISSVYTVTGPLYERDMGKLPGTQKAHTIPSAYWKVIFINNSPAVNHYAAFLFDQNTPKGADFCQFRVTVDEIEKRTGLIIWAGLPDDVQASLKSKPGVLPELMGCKN

SEQ ID NO: 164 - protein, 245 aa, synthetic construct
  REGION 1..245: note = isolated from library
DTLESIDNCAVGCPTGGSSNVSIVRHAYTLNNNSTTKFANWVAYHITKDTLASGKTRNWKTDPALNPADTLAPADYRGANAALKVDRGHQAPLASLAGVSDWESLNYLSNITPQKSDLNRGAWARLEDQERKLIDRADISSVYTVTGPLYERDMGKLPGTQKAHTIPSAYWKVIFINNSPAVNHYAAFLFDQNTPKGADFCQFRVTVDEIEKRTGLIIWAGLPDDVQASLKSKPGVLPELMGCKN

SEQ ID NO: 165 - protein, 245 aa, synthetic construct
  REGION 1..245: note = isolated from library
DTLESIDNCAVGCPTGGSSNVSIVRHAYTLNNNSTTKFANWVAYHITKDTLASGKTRNWKTDPALNPADTLAPADYRGANKALKVDRGHQAPLASLAGVSDWESLNYLSNITPQKSDLNQGAWARLEDQERKLIDRADISSVYTVTGPLYERDMGKLPGTQKAHTIPSAYWKVIFINNSPAVNHYAAFLFDQNTPKGADFCQFRVTVDEIEKRTGLIIWAGLPDDVQASLKSKPGVLPELMGCKN

SEQ ID NO: 166 - protein, 245 aa, synthetic construct
  REGION 1..245: note = isolated from library
DTLESIDNCAVGCPTGGSSNVSIVRHAYTLNNNSTTKFANWVAYHITKDTLAKGKTRNWKTDPALNPADTLAPADYRGANAALKVDRGHQAPLASLAGVSDWESLNYLSNITPQKSDLNQGAWARLEDQERKLIDRADISSVYTVTGPLYERDMGKLPGTQKAHTIPSAYWKVIFINNSPAVNHYAAFLFDQNTPKGADFCQFRVTVDEIEKRTGLIIWAGLPDDVQASLKSKPGVLPELMGCKN

SEQ ID NO: 167 - protein, 245 aa, synthetic construct
  REGION 1..245: note = isolated from library
DTLESIDNCAVGCPTGGSSNVSIVRHAYTLNNNSTTKFANWVAYHITKDTLRSGKTRNWKTDPALNPADTLAPADYRGANAALKVDRGHQAPLASLAGVSDWESLNYLSNITPQKSDLNQGAWARLEDQERKLIDRADISSVYTVTGPLYERDMGKLPGTQKAHTIPSAYWKVIFINNSPAVNHYAAFLFDQNTPKGADFCQFRVTVDEIEKRTGLIIWAGLPDDVQASLKSKPGVLPELMGCKN

SEQ ID NO: 168 - protein, 245 aa, synthetic construct
  REGION 1..245: note = isolated from library
DTLESIDNCAVGCPTGGSSNVSIVRHAYTLNNNSTTKFANWVAYHITKDTLASRKTRNWKTDPALNPADTLAPADYRGANAALKVDRGHQAPLASLAGVSDWESLNYLSNITPQKSDLNQGAWARLEDQERKLIDRADISSVYTVTGPLYERDMGKLPGTQKAHTIPSAYWKVIFINNSPAVNHYAAFLFDQNTPKGADFCQFRVTVDEIEKRTGLIIWAGLPDDVQASLKSKPGVLPELMGCKN

SEQ ID NO: 169 - protein, 245 aa, synthetic construct
  REGION 1..245: note = isolated from library
DTLESIDNCAVGCPTGGSSNVSIVRHAYTLNNNSTTKFANWVAYHITKDTLASGKTRNWKTDPALNPADTLARADYRGANAALKVDRGHQAPLASLAGVSDWESLNYLSNITPQKSDLNQGAWARLEDQERKLIDRADISSVYTVTGPLYERDMGKLPGTQKAHTIPSAYWKVIFINNSPAVNHYAAFLFDQNTPKGADFCQFRVTVDEIEKRTGLIIWAGLPDDVQASLKSKPGVLPELMGCKN

SEQ ID NO: 170 - protein, 245 aa, synthetic construct
  REGION 1..245: note = isolated from library
DTLESIDNCAVGCPTGGSSNVSIVRHAYTLNNNSTTKFANWVAYHITKDTLASGKTRNWKTDPALNPADTLAPRDYRGANAALKVDRGHQAPLASLAGVSDWESLNYLSNITPQKSDLNQGAWARLEDQERKLIDRADISSVYTVTGPLYERDMGKLPGTQKAHTIPSAYWKVIFINNSPAVNHYAAFLFDQNTPKGADFCQFRVTVDEIEKRTGLIIWAGLPDDVQASLKSKPGVLPELMGCKN

SEQ ID NO: 171 - protein, 245 aa, synthetic construct
  REGION 1..245: note = isolated from library
DTLESIDNCAVGCPTGGSSNVSIVRHAYTLNNNSTTKFANWVAYHITKDTLASGKTRNWKTDPALNPADTLAPADYRRANAALKVDRGHQAPLASLAGVSDWESLNYLSNITPQKSDLNQGAWARLEDQERKLIDRADISSVYTVTGPLYERDMGKLPGTQKAHTIPSAYWKVIFINNSPAVNHYAAFLFDQNTPKGADFCQFRVTVDEIEKRTGLIIWAGLPDDVQASLKSKPGVLPELMGCKN

SEQ ID NO: 172 - protein, 245 aa, synthetic construct
  REGION 1..245: note = isolated from library
DTLESIDNCAVGCPTGGSSNVSIVRHAYTLNNNSTTKFANWVAYHITKDTLASGKTRNWKTDPALNPADTLAPADYRGARAALKVDRGHQAPLASLAGVSDWESLNYLSNITPQKSDLNQGAWARLEDQERKLIDRADISSVYTVTGPLYERDMGKLPGTQKAHTIPSAYWKVIFINNSPAVNHYAAFLFDQNTPKGADFCQFRVTVDEIEKRTGLIIWAGLPDDVQASLKSKPGVLPELMGCKN

SEQ ID NO: 173 - protein, 245 aa, synthetic construct
  REGION 1..245: note = isolated from library
DTLESIDNCAVGCPTGGSSNVSIVRHAYTLNNNSTTKFANWVAYHITKDTLASGKTRNWKTDPALNPADTLAPADYRGANAALKVDRGHQAPLASLAGVSDWESLNYLSNITPQKSDLRQGAWARLEDQERKLIDRADISSVYTVTGPLYERDMGKLPGTQKAHTIPSAYWKVIFINNSPAVNHYAAFLFDQNTPKGADFCQFRVTVDEIEKRTGLIIWAGLPDDVQASLKSKPGVLPELMGCKN

SEQ ID NO: 174 - protein, 245 aa, synthetic construct
  REGION 1..245: note = isolated from library
DTLESIDNCAVGCPTGGSSNVSIVRHAYTLNNNSTTKFANWVAYHITKDTLASGKTRNWKTDPALNPADTLAPADYRGANAALKVDRGHQAPLASLAGVSDWESLNYLSNITPQKSDLNQGAWARLEDQERKLIDRADISSVYTVTGPLYERDMGKLPGTQKAHTIPSAYWKVIFINNSPAVNHYAAFLFDQNTRKGADFCQFRVTVDEIEKRTGLIIWAGLPDDVQASLKSKPGVLPELMGCKN

SEQ ID NO: 175 - protein, 245 aa, synthetic construct
  REGION 1..245: note = isolated from library
DTLESIDNCAVGCPTGGSSNVSIVRHAYTLNNNSTTKFANWVAYHITKDTLASGKKRNWKTDPALNPADTLAPADYRGANAALKVDRGHQAPLASLAGVSDWESLNYLSNITPQKSDLNQGAWARLEDQERKLIDRADISSVYTVTGPLYERDMGKLPGTQKAHTIPSAYWKVIFINNSPAVNHYAAFLFDQNTPKGADFCQFRVTVDEIEKRTGLIIWAGLPDDVQASLKSKPGVLPELMGCKN

SEQ ID NO: 176 - protein, 245 aa, synthetic construct
  REGION 1..245: note = isolated from library
DTLESIDNCAVGCPTGGSSNVSIVRHAYTLNNNSTTKFANWVAYHITKDTLASGKRRNWKTDPALNPADTLAPADYRGANAALKVDRGHQAPLASLAGVSDWESLNYLSNITPQKSDLNQGAWARLEDQERKLIDRADISSVYTVTGPLYERDMGKLPGTQKAHTIPSAYWKVIFINNSPAVNHYAAFLFDQNTPKGADFCQFRVTVDEIEKRTGLIIWAGLPDDVQASLKSKPGVLPELMGCKN

SEQ ID NO: 177 - protein, 245 aa, synthetic construct
  REGION 1..245: note = isolated from library
DTLESIDNCAVGCPTGGSSNVSIVRHAYTLNNNSTTKFANWVAYHITKDTLASGKTRKWKTDPALNPADTLAPADYRGANAALKVDRGHQAPLASLAGVSDWESLNYLSNITPQKSDLNQGAWARLEDQERKLIDRADISSVYTVTGPLYERDMGKLPGTQKAHTIPSAYWKVIFINNSPAVNHYAAFLFDQNTPKGADFCQFRVTVDEIEKRTGLIIWAGLPDDVQASLKSKPGVLPELMGCKN

SEQ ID NO: 178 - protein, 245 aa, synthetic construct
  REGION 1..245: note = isolated from library
DTLESIDNCAVGCPTGGSSNVSIVRHAYTLNNNSTTKFANWVAYHITKDTLASGKTRRWKTDPALNPADTLAPADYKGANAALKVDRGHQAPLASLAGVSDWESLNYLSNITPQKSDLNQGAWARLEDQERKLIDRADISSVYTVTGPLYERDMGKLPGTQKAHTIPSAYWKVIFINNSPAVNHYAAFLFDQNTPKGADFCQFRVTVDEIEKRTGLIIWAGLPDDVQASLKSKPGVLPELMGCKN

SEQ ID NO: 179 - protein, 245 aa, synthetic construct
  REGION 1..245: note = isolated from library
DTLESIDNCAVGCPTGGSSNVSIVRHAYTLNNNSTTKFANWVAYHITKDTLASGKTRNWKTDPALNPADTLAPADYKGANAALKVDRGHQAPLASLAGVSDWESLNYLSNITPQKSDLNQGAWHRLEDQERKLIDRADISSVYTVTGPLYERDMGKLPGTQKAHTIPSAYWKVIFINNSPAVNHYAAFLFDQNTPKGADFCQFRVTVDEIEKRTGLIIWAGLPDDVQASLKSKPGVLPELMGCKN

SEQ ID NO: 180 - protein, 245 aa, synthetic construct
  REGION 1..245: note = isolated from library
DTLESIDNCAVGCPTGGSSNVSIVRHAYTLNNNSTTKFANWVAYHITKDTLASGKTRNWKTDPALNPADTLAPADYKGANAALKVDRGHQAPLASLAGVSDWESLNYLSNITPQKSDLNQGAWKRLEDQERKLIDRADISSVYTVTGPLYERDMGKLPGTQKAHTIPSAYWKVIFINNSPAVNHYAAFLFDQNTPKGADFCQFRVTVDEIEKRTGLIIWAGLPDDVQASLKSKPGVLPELMGCKN

SEQ ID NO: 181 - protein, 245 aa, synthetic construct
  REGION 1..245: note = isolated from library
DTLESIDNCAVGCPTGGSSNVSIVRHAYTLNNNSTTKFANWVAYHITKDTGASGKTRNWKTDPALNPADTLAPADYKGANAALKVDRGHQAPLASLAGVSDWESLNYLSNITPQKSDLNQGAWKRLEDQERKLIDRADISSVYTVTGPLYERDMGKLPGTQKAHTIPSAYWKVIFINNSPAVNHYAAFLFDQNTPKGADFCQFRVTVDEIEKRTGLIIWAGLPDDVQASLKSKPGVLPELMGCKN

SEQ ID NO: 182 - protein, 245 aa, synthetic construct
  REGION 1..245: note = isolated from library
DTLESIDNCAVGCPTGGSSNVSIVRHAYTLNNNSTTKFANWVAYHITKDTGASGKTRNWKTDPALNPADTLAPADYKGANAALKVDRGHQAPLASLAGVSDWESLNYLSNITPQKSDLNQGAWRRLEDQERKLIDRADISSVYTVTGPLYERDMGKLPGTQKAHTIPSAYWKVIFINNSPAVNHYAAFLFDQNTPKGADFCQFRVTVDEIEKRTGLIIWAGLPDDVQASLKSKPGVLPELMGCKN

SEQ ID NO: 183 - protein, 245 aa, synthetic construct
  REGION 1..245: note = isolated from library
DTLESIDNCAVGCPTGGSSNVSIVRHAYTLNNNSTTKFANWVAYHITKDTGASGKTRNWKTDPALNPADTLAPADYKGANAALKVDRGHQAPLASLAGVSDWESLNYLSNITPQKSDLNQGAWHRLEDQERKLIDRADISSVYTVTGPLYERDMGKLPGTQKAHTIPSAYWKVIFINNSPAVNHYAAFLFDQNTPKGADFCQFRVTVDEIEKRTGLIIWAGLPDDVQASLKSKPGVLPELMGCKN

SEQ ID NO: 184 - protein, 245 aa, synthetic construct
  REGION 1..245: note = isolated from library
DTLESIDNCAVGCPTGGSSNVSIVRHAYTLNNNSTTKFANWVAYHITKDTGASGKTRNWKTDPALNPADTLAPADYRGANAALKVDRGHQAPLASLAGVSDWESLNYLSNITPQKSDLNQGAWRRLEDQERKLIDRADISSVYTVTGPLYERDMGKLPGTQKAHTIPSAYWKVIFINNSPAVNHYAAFLFDQNTPKGADFCQFRVTVDEIEKRTGLIIWAGLPDDVQASLKSKPGVLPELMGCKN

SEQ ID NO: 185 - protein, 245 aa, synthetic construct
  REGION 1..245: note = isolated from library
DTLESIDNCAVGCPTGGSSNVSIVRHAYTLNNNSTTKFANWVAYHITKDTGASGKTRNWKTDPALNPADTLAPADYRGANAALKVDRGHQAPLASLAGVSDWESLNYLSNITPQKSDLNQGAWKRLEDQERKLIDRADISSVYTVTGPLYERDMGKLPGTQKAHTIPSAYWKVIFINNSPAVNHYAAFLFDQNTPKGADFCQFRVTVDEIEKRTGLIIWAGLPDDVQASLKSKPGVLPELMGCKN

SEQ ID NO: 186 - protein, 245 aa, synthetic construct
  REGION 1..245: note = isolated from library
DTLESIDNCAVGCPTGGSSNVSIVRHAYTLNNNSTTKFANWVAYHITKDTGASGKTRNWKTDPALNPADTLAPADYRGANAALKVDRGHQAPLASLAGVSDWESLNYLSNITPQKSDLNQGAWHRLEDQERKLIDRADISSVYTVTGPLYERDMGKLPGTQKAHTIPSAYWKVIFINNSPAVNHYAAFLFDQNTPKGADFCQFRVTVDEIEKRTGLIIWAGLPDDVQASLKSKPGVLPELMGCKN

SEQ ID NO: 187 - protein, 245 aa, synthetic construct
  REGION 1..245: note = isolated from library
DTLESIDNCAVGCPTGGSSNVSIVRHAYTLNNNSTTKFANWVAYHITKDTLASGKTRNWKTDPALNPADTLAPADYHGANAALKVDRGHQAPLASLAGVSDWESLNYLSNITPQKSDLNQGAWRRLEDQERKLIDRADISSVYTVTGPLYERDMGKLPGTQKAHTIPSAYWKVIFINNSPAVNHYAAFLFDQNTPKGADFCQFRVTVDEIEKRTGLIIWAGLPDDVQASLKSKPGVLPELMGCKN

SEQ ID NO: 188 - protein, 245 aa, synthetic construct
  REGION 1..245: note = isolated from library
DTLESIDNCAVGCPTGGSSNVSIVRHAYTLNNNSTTKFANWVAYHITKDTLASGKTRNWKTDPALNPADTLAPADYHGANAALKVDRGHQAPLASLAGVSDWESLNYLSNITPQKSDLNQGAWKRLEDQERKLIDRADISSVYTVTGPLYERDMGKLPGTQKAHTIPSAYWKVIFINNSPAVNHYAAFLFDQNTPKGADFCQFRVTVDEIEKRTGLIIWAGLPDDVQASLKSKPGVLPELMGCKN

SEQ ID NO: 189 - protein, 245 aa, synthetic construct
  REGION 1..245: note = isolated from library
DTLESIDNCAVGCPTGGSSNVSIVRHAYTLNNNSTTKFANWVAYHITKDTLASGKTRNWKTDPALNPADTLAPADYHGANAALKVDRGHQAPLASLAGVSDWESLNYLSNITPQKSDLNQGAWHRLEDQERKLIDRADISSVYTVTGPLYERDMGKLPGTQKAHTIPSAYWKVIFINNSPAVNHYAAFLFDQNTPKGADFCQFRVTVDEIEKRTGLIIWAGLPDDVQASLKSKPGVLPELMGCKN

SEQ ID NO: 190 - protein, 245 aa, synthetic construct
  REGION 1..245: note = isolated from library
DTLESIDNCAVGCPTGGSSNVSIVRHAYTLNNNSTTKFANWVAYHITKDTGASGKTRNWKTDPALNPADTLAPADYHGANAALKVDRGHQAPLASLAGVSDWESLNYLSNITPQKSDLNQGAWRRLEDQERKLIDRADISSVYTVTGPLYERDMGKLPGTQKAHTIPSAYWKVIFINNSPAVNHYAAFLFDQNTPKGADFCQFRVTVDEIEKRTGLIIWAGLPDDVQASLKSKPGVLPELMGCKN

SEQ ID NO: 191 - protein, 245 aa, synthetic construct
  REGION 1..245: note = isolated from library
DTLESIDNCAVGCPTGGSSNVSIVRHAYTLNNNSTTKFANWVAYHITKDTGASGKTRNWKTDPALNPADTLAPADYHGANAALKVDRGHQAPLASLAGVSDWESLNYLSNITPQKSDLNQGAWKRLEDQERKLIDRADISSVYTVTGPLYERDMGKLPGTQKAHTIPSAYWKVIFINNSPAVNHYAAFLFDQNTPKGADFCQFRVTVDEIEKRTGLIIWAGLPDDVQASLKSKPGVLPELMGCKN

SEQ ID NO: 192 - protein, 245 aa, synthetic construct
  REGION 1..245: note = isolated from library
DTLESIDNCAVGCPTGGSSNVSIVRHAYTLNNNSTTKFANWVAYHITKDTGASGKTRNWKTDPALNPADTLAPADYHGANAALKVDRGHQAPLASLAGVSDWESLNYLSNITPQKSDLNQGAWHRLEDQERKLIDRADISSVYTVTGPLYERDMGKLPGTQKAHTIPSAYWKVIFINNSPAVNHYAAFLFDQNTPKGADFCQFRVTVDEIEKRTGLIIWAGLPDDVQASLKSKPGVLPELMGCKN

SEQ ID NO: 193 - protein, 245 aa, synthetic construct
  REGION 1..245: note = isolated from library
DTLESIDNCAVGCPTGGSSNVSIVRHAYTLNNNSTTKFANWVAYHITKDTAASGKTRNWKTDPALNPADTLAPADYRGANAALKVDRGHQAPLASLAGVSDWESLNYLSNITPQKSDLNQGAWKRLEDQERKLIDRADISSVYTVTGPLYERDMGKLPGTQKAHTIPSAYWKVIFINNSPAVNHYAAFLFDQNTPKGADFCQFRVTVDEIEKRTGLIIWAGLPDDVQASLKSKPGVLPELMGCKN

SEQ ID NO: 194 - protein, 245 aa, synthetic construct
  REGION 1..245: note = isolated from library
DTLESIDNCAVGCPTGGSSNVSIVRHAYTLNNNSTTKFANWVAYHITKDTVASGKTRNWKTDPALNPADTLAPADYRGANAALKVDRGHQAPLASLAGVSDWESLNYLSNITPQKSDLNQGAWKRLEDQERKLIDRADISSVYTVTGPLYERDMGKLPGTQKAHTIPSAYWKVIFINNSPAVNHYAAFLFDQNTPKGADFCQFRVTVDEIEKRTGLIIWAGLPDDVQASLKSKPGVLPELMGCKN

SEQ ID NO: 195 - protein, 245 aa, synthetic construct
  REGION 1..245: note = isolated from library
DTLESIDNCAVGCPTGGSSNVSIVRHAYTLNNNSTTKFANWVAYHITKDTIASGKTRNWKTDPALNPADTLAPADYRGANAALKVDRGHQAPLASLAGVSDWESLNYLSNITPQKSDLNQGAWKRLEDQERKLIDRADISSVYTVTGPLYERDMGKLPGTQKAHTIPSAYWKVIFINNSPAVNHYAAFLFDQNTPKGADFCQFRVTVDEIEKRTGLIIWAGLPDDVQASLKSKPGVLPELMGCKN